European Patent Application EP 4 155 319 A1, published March 29, 2023. Title: 4-1BB BINDING PROTEIN AND APPLICATION THEREOF. Applicant: NONA BIOSCIENCES (SUZHOU) CO., LTD. Application 21832365.7. The sequence listing filed with the application follows.

SEQUENCE LISTING (382 sequences)

SEQ ID NO: 1 - protein, 25 aa, Artificial Sequence [sequence omitted]

SEQ ID NO: 2 - protein, 25 aa, Artificial Sequence
  PR000196 HFWR1 Chothia
EVQLLESGGGLVQRGGSLRLSCAAS

SEQ ID NO: 3 - protein, 25 aa, Artificial Sequence [sequence omitted]

SEQ ID NO: 4 - protein, 25 aa, Artificial Sequence
  PR000483 HFWR1 Chothia
EVQLVQSGAEVKKPGESLRISCKGS

SEQ ID NO: 5 - protein, 25 aa, Artificial Sequence
  PR001758 HFWR1 Chothia, PR001781 HFWR1 Chothia
EVQLLESGGGLVQLGGSLRLSCAAS

SEQ ID NO: 6 - protein, 25 aa, Artificial Sequence
  PR001759 HFWR1 Chothia, PR001764 HFWR1 Chothia, PR001766 HFWR1 Chothia
EVQLLESGGGLVQPGGSLRLSCAAS

SEQ ID NO: 7 - protein, 25 aa, Artificial Sequence
  PR001760 HFWR1 Chothia
EVQLVESGGGVVQPGGSLRLSCAAS

SEQ ID NO: 8 - protein, 25 aa, Artificial Sequence
  PR001763 HFWR1 Chothia, PR001830 HFWR1 Chothia
EVQLLESGGGLVQPGGSLRLSCTAS

SEQ ID NO: 9 - protein, 25 aa, Artificial Sequence
  PR001767 HFWR1 Chothia
EVQLVETGGGLIQPGGSLRLSCAAS

SEQ ID NO: 10 - protein, 25 aa, Artificial Sequence
  PR001775 HFWR1 Chothia
EVQLLESGGGLVQSGGSLRLSCAAS

SEQ ID NO: 11 - protein, 25 aa, Artificial Sequence
  PR001780 HFWR1 Chothia
EVQLLESGGGLIQPGGSLRLSCAAS

SEQ ID NO: 12 - protein, 25 aa, Artificial Sequence
  PR001831 HFWR1 Chothia
EVQLVESGGGVIQPGGSLRLSCEAS

SEQ ID NO: 13 - protein, 25 aa, Artificial Sequence
  PR001837 HFWR1 Chothia
EVQLLESGGGLVQPGGSLRLSCEAS

SEQ ID NO: 14 - protein, 7 aa, Artificial Sequence
  PR000151 HCDR1 Chothia
GFTFSDS

SEQ ID NO: 15 - protein, 7 aa, Artificial Sequence
  PR000196 HCDR1 Chothia, PR000265 HCDR1 Chothia, PR001759 HCDR1 Chothia
GFTFSSY

SEQ ID NO: 16 - protein, 7 aa, Artificial Sequence
  PR000197 HCDR1 Chothia, PR000447 HCDR1 Chothia, PR000448 HCDR1 Chothia
GGSFSGY

SEQ ID NO: 17 - protein, 7 aa, Artificial Sequence
  PR000210 HCDR1 Chothia
GFNIKDT

SEQ ID NO: 18 - protein, 7 aa, Artificial Sequence
  PR000483 HCDR1 Chothia
GYSFSTY

SEQ ID NO: 19 - protein, 7 aa, Artificial Sequence
  PR001758 HCDR1 Chothia
GFTFSRY

SEQ ID NO: 20 - protein, 7 aa, Artificial Sequence
  PR001760 HCDR1 Chothia, PR001763 HCDR1 Chothia, PR001768 HCDR1 Chothia
GFTFSNY

SEQ ID NO: 21 - protein, 7 aa, Artificial Sequence
  PR001767 HCDR1 Chothia
GFTVSSN

SEQ ID NO: 22 - protein, 7 aa, Artificial Sequence
  PR001774 HCDR1 Chothia, PR001780 HCDR1 Chothia
GFTFSSF

SEQ ID NO: 23 - protein, 7 aa, Artificial Sequence
  PR001834 HCDR1 Chothia
GFTFSGY

SEQ ID NO: 24 - protein, 7 aa, Artificial Sequence
  PR001836 HCDR1 Chothia
GFIFSNF

SEQ ID NO: 25 - protein, 19 aa, Artificial Sequence
  PR000151 HFWR2 Chothia
WIHWVRQAPGKGLEWVAWI

SEQ ID NO: 26 - protein, 19 aa, Artificial Sequence
  PR000196 HFWR2 Chothia
AMTWVRQAPGKGLEWVSAI

SEQ ID NO: 27 - protein, 19 aa, Artificial Sequence
  PR000197 HFWR2 Chothia, PR000447 HFWR2 Chothia, PR000448 HFWR2 Chothia
YWSWIRQPPGKGLEWIGEI

SEQ ID NO: 28 - protein, 19 aa, Artificial Sequence
  PR000210 HFWR2 Chothia
YIHWVRQAPGKGLEWVARI

SEQ ID NO: 29 - protein, 19 aa, Artificial Sequence
  PR000265 HFWR2 Chothia
WMSWVRQAPGKGLEWVANI

SEQ ID NO: 30 - protein, 19 aa, Artificial Sequence
  PR000483 HFWR2 Chothia
WISWVRQMPGKGLEWMGKI

SEQ ID NO: 31 - protein, 19 aa, Artificial Sequence
  PR000628 HFWR2 Chothia
YWSWIRQSPEKGLEWIGEI

SEQ ID NO: 32 - protein, 19 aa, Artificial Sequence
  PR001758 HFWR2 Chothia, PR001760 HFWR2 Chothia, PR001781 HFWR2 Chothia
AMTWVRQAPEKGLEWVSSI

SEQ ID NO: 33 - protein, 19 aa, Artificial Sequence
  PR001759 HFWR2 Chothia
AMSWFRQPPETGLQWVSSI

SEQ ID NO: 34 - protein, 19 aa, Artificial Sequence
  PR001763 HFWR2 Chothia, PR001830 HFWR2 Chothia, PR001831 HFWR2 Chothia
AMSWVRQAPEKGLEWVSSI

SEQ ID NO: 35 - protein, 19 aa, Artificial Sequence
  PR001764 HFWR2 Chothia, PR001776 HFWR2 Chothia
AMSWVRQAPEKGLEWVSAI

SEQ ID NO: 36 - protein, 19 aa, Artificial Sequence
  PR001766 HFWR2 Chothia
AMSWGRQAPGKGLEWVSSI

SEQ ID NO: 37 - protein, 19 aa, Artificial Sequence
  PR001767 HFWR2 Chothia
YMSWVRQAPGKGLEWVSVI

SEQ ID NO: 38 - protein, 19 aa, Artificial Sequence
  PR001768 HFWR2 Chothia
AMTWVRQAPGKGLEWVSSI

SEQ ID NO: 39 - protein, 19 aa, Artificial Sequence
  PR001771 HFWR2 Chothia
AMTWVRQPPGKGLEWVSSI

SEQ ID NO: 40 - protein, 19 aa, Artificial Sequence
  PR001774 HFWR2 Chothia
AMTWVRQAPEKGLEWVSTI

SEQ ID NO: 41 - protein, 19 aa, Artificial Sequence
  PR001775 HFWR2 Chothia
AMSWVRQAPGKGLEWVSAI

SEQ ID NO: 42 - protein, 19 aa, Artificial Sequence
  PR001780 HFWR2 Chothia
AMTWVRQAPGKGLEWVSTI

SEQ ID NO: 43 - protein, 19 aa, Artificial Sequence
  PR001834 HFWR2 Chothia
AMTWVRQPPEKGLEWVSSI

SEQ ID NO: 44 - protein, 19 aa, Artificial Sequence
  PR001836 HFWR2 Chothia
AMTWVRQPPEKGLKWVSSI

SEQ ID NO: 45 - protein, 19 aa, Artificial Sequence
  PR001838 HFWR2 Chothia, PR004469 HFWR2 Chothia
AMSWFRQPPETGLKWVSSI

SEQ ID NO: 46 - protein, 19 aa, Artificial Sequence
  PR001840 HFWR2 Chothia
WMHWVRQAPGKGLVWVSRI

SEQ ID NO: 47 - protein, 19 aa, Artificial Sequence
  PR001842 HFWR2 Chothia
AMSWGRQAPGKGLEWVSAI

SEQ ID NO: 48 - protein, 6 aa, Artificial Sequence
  PR000151 HCDR2 Chothia
SPYGGS

SEQ ID NO: 49 - protein, 6 aa, Artificial Sequence
  PR000196 HCDR2 Chothia, PR001781 HCDR2 Chothia
SGSGGN

SEQ ID NO: 50 - protein, 5 aa, Artificial Sequence
  PR000197 HCDR2 Chothia
NHSGS

SEQ ID NO: 51 - protein, 6 aa, Artificial Sequence
  PR000210 HCDR2 Chothia
YPTNGY

SEQ ID NO: 52 - protein, 6 aa, Artificial Sequence
  PR000265 HCDR2 Chothia
KQEGSE

SEQ ID NO: 53 - protein, 5 aa, Artificial Sequence
  PR000447 HCDR2 Chothia
IHSGS

SEQ ID NO: 54 - protein, 5 aa, Artificial Sequence
  PR000448 HCDR2 Chothia, PR000980 HCDR2 Chothia
QHSGS

SEQ ID NO: 55 - protein, 6 aa, Artificial Sequence
  PR000483 HCDR2 Chothia
YPGDSY

SEQ ID NO: 56 - protein, 5 aa, Artificial Sequence
  PR000628 HCDR2 Chothia
NHGGY

SEQ ID NO: 57 - protein, 6 aa, Artificial Sequence
  PR001758 HCDR2 Chothia
SGSGDD

SEQ ID NO: 58 - protein, 6 aa, Artificial Sequence
  PR001759 HCDR2 Chothia
GGSGGD

SEQ ID NO: 59 - protein, 6 aa, Artificial Sequence
  PR001760 HCDR2 Chothia
SGSGVS

SEQ ID NO: 60 - protein, 6 aa, Artificial Sequence
  PR001763 HCDR2 Chothia, PR001766 HCDR2 Chothia, PR001771 HCDR2 Chothia
SGSGGS

SEQ ID NO: 61 - protein, 6 aa, Artificial Sequence
  PR001764 HCDR2 Chothia
SGGGGS

SEQ ID NO: 62 - protein, 5 aa, Artificial Sequence
  PR001767 HCDR2 Chothia
YSDGS

SEQ ID NO: 63 - protein, 6 aa, Artificial Sequence
  PR001768 HCDR2 Chothia, PR001831 HCDR2 Chothia
SGSGDS

SEQ ID NO: 64 - protein, 6 aa, Artificial Sequence
  PR001774 HCDR2 Chothia
SGSGDT

SEQ ID NO: 65 - protein, 6 aa, Artificial Sequence
  PR001776 HCDR2 Chothia
SSSGGS

SEQ ID NO: 66 - protein, 6 aa, Artificial Sequence
  PR001780 HCDR2 Chothia
SGSGDN

SEQ ID NO: 67 - protein, 6 aa, Artificial Sequence
  PR001834 HCDR2 Chothia
SGSGNN

SEQ ID NO: 68 - protein, 6 aa, Artificial Sequence
  PR001836 HCDR2 Chothia
NGSGFN

SEQ ID NO: 69 - protein, 6 aa, Artificial Sequence
  PR001838 HCDR2 Chothia
DGSGGD

SEQ ID NO: 70 - protein, 6 aa, Artificial Sequence
  PR001840 HCDR2 Chothia
NSDGSS

SEQ ID NO: 71 - protein, 6 aa, Artificial Sequence
  PR004469 HCDR2 Chothia, PR007381 HCDR2 Chothia
DASGGD

SEQ ID NO: 72 - protein, 41 aa, Artificial Sequence
  PR000151 HFWR3 Chothia
TYYADSVKGRFTISADTSKNTAYLQMNSLRAEDTAVYYCAR

SEQ ID NO: 73 - protein, 41 aa, Artificial Sequence
  PR000196 HFWR3 Chothia
TYYADSVRGRFTISRDNSKNTLYLQMNSLRAEDTAVYFCAK

SEQ ID NO: 74 - protein, 41 aa, Artificial Sequence
  PR000197 HFWR3 Chothia, PR000447 HFWR3 Chothia, PR000448 HFWR3 Chothia
TDSNPSLKGRVTFSVDTSKNQFSLKLNSVTAADTAVYYCAR

SEQ ID NO: 75 - protein, 41 aa, Artificial Sequence
  PR000210 HFWR3 Chothia
TRYADSVKGRFTISADTSKNTAYLQMNSLRAEDTAVYYCSR

SEQ ID NO: 76 - protein, 41 aa, Artificial Sequence
  PR000265 HFWR3 Chothia
KYYVDSVKGRFTISRDNAKNSLYLQMNSLRAEDTAVYYCAR

SEQ ID NO: 77 - protein, 41 aa, Artificial Sequence
  PR000483 HFWR3 Chothia
TNYSPSFQGQVTISADKSISTAYLQWSSLKASDTAMYYCAR

SEQ ID NO: 78 - protein, 41 aa, Artificial Sequence
  PR000628 HFWR3 Chothia
VTYNPSLESRVTISVDTSKNQFSLKLSSVTAADTAVYYCAR

SEQ ID NO: 79 - protein, 41 aa, Artificial Sequence
  PR001758 HFWR3 Chothia
TYYGDSVKGRFTISRDNSQNTVYLQMNSLRAEDTAVYFCAK

SEQ ID NO: 80 - protein, 41 aa, Artificial Sequence
  PR001759 HFWR3 Chothia, PR001766 HFWR3 Chothia, PR001768 HFWR3 Chothia
TYYADSVKGRFTISRDNSKNTLYLQMNSLRAEDTAVYYCAK

SEQ ID NO: 81 - protein, 41 aa, Artificial Sequence
  PR001760 HFWR3 Chothia
TYYADSVKGRFTISRDNSKNTLYLQMTRLTAEDTAVYFCAK

SEQ ID NO: 82 - protein, 41 aa, Artificial Sequence
  PR001763 HFWR3 Chothia
TFYADSVKGRFTISRDNSKNTLYLQMNRLTAEDTAVYYCAK

SEQ ID NO: 83 - protein, 41 aa, Artificial Sequence
  PR001764 HFWR3 Chothia
TYYADSVKGRFTISRDNSKNTLYLQMDSLKAEDTAVYYCAK

SEQ ID NO: 84 - protein, 41 aa, Artificial Sequence
  PR001767 HFWR3 Chothia
TYYADSVKGRFTISRDNSKNTLYLQMNSLRAEDTAVYYCAR

SEQ ID NO: 85 - protein, 41 aa, Artificial Sequence
  PR001774 HFWR3 Chothia
TYYADSVKGRFTISRDSSKNTLYLQMNSLRAEDSAVYFCAK

SEQ ID NO: 86 - protein, 41 aa, Artificial Sequence
  PR001775 HFWR3 Chothia
TDYADSVKGRFTISRDNSTNTLYLQMNSLRAEDTAVYYCAK

SEQ ID NO: 87 - protein, 41 aa, Artificial Sequence
  PR001780 HFWR3 Chothia
TYYADSVKGRFTISRDNSKNTLYLQMNSLRAEDTAVYFCAK

SEQ ID NO: 88 - protein, 41 aa, Artificial Sequence
  PR001830 HFWR3 Chothia, PR001833 HFWR3 Chothia
TFYADSVKGRFTISRDNSKNTLYLQMNSLRAEDTAVYFCAK

SEQ ID NO: 89 - protein, 41 aa, Artificial Sequence
  PR001831 HFWR3 Chothia
TYYADSVKGRFTISRDNSKNTLYLQMNSLRAEDTAGYHCAK

SEQ ID NO: 90 - protein, 41 aa, Artificial Sequence
  PR001834 HFWR3 Chothia, PR001837 HFWR3 Chothia
TFYADSVKGRFTISRDNSKNTLYLQMNSLRAEDTAVYYCAK

SEQ ID NO: 91 - protein, 41 aa, Artificial Sequence
  PR001836 HFWR3 Chothia
TYYTDSVKGRFTISRDNSRNTLYLQMNRLTAEDTAVYFCAK

SEQ ID NO: 92 - protein, 41 aa, Artificial Sequence
  PR001840 HFWR3 Chothia
TSYADSVQGRFTISRDNAKNTLYLQMNSLRAEDTAVYYCVR

SEQ ID NO: 93 - protein, 41 aa, Artificial Sequence
  PR001842 HFWR3 Chothia
TYYADSVKGRFTISRDNSKNTLYLHMNSLRAEDTAVYYCAK

SEQ ID NO: 94 - protein, 9 aa, Artificial Sequence
  PR000151 HCDR3 Chothia
RHWPGGFDY

SEQ ID NO: 95 - protein, 20 aa, Artificial Sequence
  PR000196 HCDR3 Chothia
EAYHYGSGSYYDDYYYGMDV

SEQ ID NO: 96 - protein, 7 aa, Artificial Sequence
  PR000197 HCDR3 Chothia, PR000447 HCDR3 Chothia, PR000448 HCDR3 Chothia
LTGPFDY

SEQ ID NO: 97 - protein, 11 aa, Artificial Sequence
  PR000210 HCDR3 Chothia
WGGDGFYAMDY

SEQ ID NO: 98 - protein, 10 aa, Artificial Sequence
  PR000265 HCDR3 Chothia
DRAVAGAFDI

SEQ ID NO: 99 - protein, 7 aa, Artificial Sequence
  PR000483 HCDR3 Chothia
GYGIFDY

SEQ ID NO: 100 - protein, 13 aa, Artificial Sequence
  PR000628 HCDR3 Chothia
DYGPGNYDWYFDL

SEQ ID NO: 101 - protein, 15 aa, Artificial Sequence
  PR001758 HCDR3 Chothia
EKAGTTGDYYYNVDV

SEQ ID NO: 102 - protein, 15 aa, Artificial Sequence
  PR001759 HCDR3 Chothia
EGSNGTDDNYYDVDV

SEQ ID NO: 103 - protein, 15 aa, Artificial Sequence
  PR001760 HCDR3 Chothia, PR001830 HCDR3 Chothia, PR001836 HCDR3 Chothia
EGSSETDDHYYNVDV

SEQ ID NO: 104 - protein, 15 aa, Artificial Sequence
  PR001763 HCDR3 Chothia, PR001831 HCDR3 Chothia
EGSNGTDDYHYDIDV

SEQ ID NO: 105 - protein, 15 aa, Artificial Sequence
  PR001764 HCDR3 Chothia, PR001834 HCDR3 Chothia, PR001837 HCDR3 Chothia
EGTTETDDYHYNMDV

SEQ ID NO: 106 - protein, 15 aa, Artificial Sequence
  PR001766 HCDR3 Chothia
EKTGTTGDYYYDMDV

SEQ ID NO: 107 - protein, 18 aa, Artificial Sequence
  PR001767 HCDR3 Chothia
DRYYGSGNYPTAYYGMDV

SEQ ID NO: 108 - protein, 15 aa, Artificial Sequence
  PR001768 HCDR3 Chothia, PR001771 HCDR3 Chothia
EGTGTTSDYYYNVDV

SEQ ID NO: 109 - protein, 15 aa, Artificial Sequence
  PR001774 HCDR3 Chothia
EATAMASDYYYGVDV

SEQ ID NO: 110 - protein, 14 aa, Artificial Sequence
  PR001775 HCDR3 Chothia
ERAYDYSNYVDFDY

SEQ ID NO: 111 - protein, 16 aa, Artificial Sequence
  PR001776 HCDR3 Chothia
DGVTTPSYYYYYDMDV

SEQ ID NO: 112 - protein, 15 aa, Artificial Sequence
  PR001780 HCDR3 Chothia
EDTAVASDYYYNIDV

SEQ ID NO: 113 - protein, 15 aa, Artificial Sequence
  PR001781 HCDR3 Chothia
ERTGTTGDYYYNVDV

SEQ ID NO: 114 - protein, 15 aa, Artificial Sequence
  PR001833 HCDR3 Chothia
EGATETDDYHFNTDV

SEQ ID NO: 115 - protein, 15 aa, Artificial Sequence
  PR001838 HCDR3 Chothia, PR004469 HCDR3 Chothia, PR007381 HCDR3 Chothia
EGSHGTDDSHYDVDV

SEQ ID NO: 116 - protein, 14 aa, Artificial Sequence
  PR001840 HCDR3 Chothia
KGSSSYYHYSIEDD

SEQ ID NO: 117 - protein, 15 aa, Artificial Sequence
  PR001842 HCDR3 Chothia
EKVATTGDYYYDMDV

SEQ ID NO: 118 - protein, 11 aa, Artificial Sequence
  PR000151 HFWR4 Chothia, PR000197 HFWR4 Chothia, PR000210 HFWR4 Chothia
WGQGTLVTVSS

SEQ ID NO: 119 - protein, 11 aa, Artificial Sequence
  PR000196 HFWR4 Chothia, PR001758 HFWR4 Chothia, PR001759 HFWR4 Chothia
WGQGTTVTVSS

SEQ ID NO: 120 - protein, 11 aa, Artificial Sequence
  PR000265 HFWR4 Chothia, PR007295 HFWR4 Chothia
WGQGTMVTVSS

SEQ ID NO: 121 - protein, 11 aa, Artificial Sequence
  PR000628 HFWR4 Chothia
WGRGTLVTVSS

SEQ ID NO: 122 - protein, 11 aa, Artificial Sequence
  PR001767 HFWR4 Chothia
RGQGTTVTVSS

SEQ ID NO: 123 - protein, 11 aa, Artificial Sequence
  PR001831 HFWR4 Chothia
WGQGTSVTVSS

SEQ ID NO: 124 - protein, 23 aa, Artificial Sequence
  PR000151 LFWR1 Chothia, PR000210 LFWR1 Chothia
DIQMTQSPSSLSASVGDRVTITC

SEQ ID NO: 125 - protein, 23 aa, Artificial Sequence
  PR000196 LFWR1 Chothia
DIVMTQSPLSLPVTPGEPASISC

SEQ ID NO: 126 - protein, 23 aa, Artificial Sequence
  PR000197 LFWR1 Chothia
EFVMTQSPATLSVSPGERATLSC

SEQ ID NO: 127 - protein, 23 aa, Artificial Sequence
  PR000265 LFWR1 Chothia
DIQMTQSPSTLSASVGDRVTVTC

SEQ ID NO: 128 - protein, 23 aa, Artificial Sequence
  PR000447 LFWR1 Chothia, PR000448 LFWR1 Chothia, PR000980 LFWR1 Chothia
EIVMTQSPATLSVSPGERATLSC

SEQ ID NO: 129 - protein, 22 aa, Artificial Sequence
  PR000483 LFWR1 Chothia
SYELTQPPSVSVSPGQTASITC

SEQ ID NO: 130 - protein, 23 aa, Artificial Sequence
  PR000628 LFWR1 Chothia
EIVLTQSPATLSLSPGERATLSC

SEQ ID NO: 131 - protein, 11 aa, Artificial Sequence
  PR000151 LCDR1 Chothia
RASQDVSTAVA

SEQ ID NO: 132 - protein, 16 aa, Artificial Sequence
  PR000196 LCDR1 Chothia
RSSQSLLHSNGYNYLD

SEQ ID NO: 133 - protein, 11 aa, Artificial Sequence
  PR000197 LCDR1 Chothia, PR000447 LCDR1 Chothia, PR000448 LCDR1 Chothia
RASQSISSILA

SEQ ID NO: 134 - protein, 11 aa, Artificial Sequence
  PR000210 LCDR1 Chothia
RASQDVNTAVA

SEQ ID NO: 135 - protein, 11 aa, Artificial Sequence
  PR000265 LCDR1 Chothia
RASQSIYIWLA

SEQ ID NO: 136 - protein, 11 aa, Artificial Sequence
  PR000483 LCDR1 Chothia
SGDNIGDQYAH

SEQ ID NO: 137 - protein, 11 aa, Artificial Sequence
  PR000628 LCDR1 Chothia
RASQSVSSYLA

SEQ ID NO: 138 - protein, 15 aa, Artificial Sequence
  PR000151 LFWR2 Chothia, PR000210 LFWR2 Chothia
WYQQKPGKAPKLLIY

SEQ ID NO: 139 - protein, 15 aa, Artificial Sequence
  PR000196 LFWR2 Chothia
WYLQKPGQSPQLLIF

SEQ ID NO: 140 - protein, 15 aa, Artificial Sequence
  PR000197 LFWR2 Chothia, PR000447 LFWR2 Chothia, PR000448 LFWR2 Chothia
WYQQKPGQAPRLLIY

SEQ ID NO: 141 - protein, 15 aa, Artificial Sequence
  PR000265 LFWR2 Chothia
WYQQKPGKAPNLLIY

SEQ ID NO: 142 - protein, 15 aa, Artificial Sequence
  PR000483 LFWR2 Chothia
WYQQKPGQSPVLVIY

SEQ ID NO: 143 - protein, 7 aa, Artificial Sequence
  PR000151 LCDR2 Chothia, PR000210 LCDR2 Chothia
SASFLYS

SEQ ID NO: 144 - protein, 7 aa, Artificial Sequence
  PR000196 LCDR2 Chothia
LGSNRAS

SEQ ID NO: 145 - protein, 7 aa, Artificial Sequence
  PR000197 LCDR2 Chothia, PR000447 LCDR2 Chothia, PR000448 LCDR2 Chothia
GASTRAT

SEQ ID NO: 146 - protein, 7 aa, Artificial Sequence
  PR000265 LCDR2 Chothia
KASSLET

SEQ ID NO: 147 - protein, 7 aa, Artificial Sequence
  PR000483 LCDR2 Chothia
QDKNRPS

SEQ ID NO: 148 - protein, 7 aa, Artificial Sequence
  PR000628 LCDR2 Chothia
DASNRAT

SEQ ID NO: 149 - protein, 32 aa, Artificial Sequence
  PR000151 LFWR3 Chothia
GVPSRFSGSGSGTDFTLTISSLQPEDFATYYC

SEQ ID NO: 150 - protein, 32 aa, Artificial Sequence
  PR000196 LFWR3 Chothia
GVPDRFSGSGSGTDFTLKISRVEAEDVGVYYC

SEQ ID NO: 151 - protein, 32 aa, Artificial Sequence
  PR000197 LFWR3 Chothia, PR000447 LFWR3 Chothia, PR000448 LFWR3 Chothia
GIPARFSGSGSGTEFTLTISSLQSEDFAVYYC

SEQ ID NO: 152 - protein, 32 aa, Artificial Sequence
  PR000210 LFWR3 Chothia
GVPSRFSGSRSGTDFTLTISSLQPEDFATYYC

SEQ ID NO: 153 - protein, 32 aa, Artificial Sequence
  PR000265 LFWR3 Chothia
GVPSRFSGSGSGTEFTLTISSLQPDDFATYYC

SEQ ID NO: 154 - protein, 32 aa, Artificial Sequence
  PR000483 LFWR3 Chothia
GIPERFSGSNSGNTATLTISGTQAMDEADYYC

SEQ ID NO: 155 - protein, 32 aa, Artificial Sequence
  PR000628 LFWR3 Chothia
GIPARFSGSGSGTDFTLTISSLEPEDFAVYYC

SEQ ID NO: 156 - protein, 9 aa, Artificial Sequence
  PR000151 LCDR3 Chothia
QQYLYHPAT

SEQ ID NO: 157 - protein, 9 aa, Artificial Sequence
  PR000196 LCDR3 Chothia
MQALQTPLT

SEQ ID NO: 158 - protein, 9 aa, Artificial Sequence
  PR000197 LCDR3 Chothia, PR000447 LCDR3 Chothia, PR000448 LCDR3 Chothia
QQYYNWPLT

SEQ ID NO: 159 - protein, 9 aa, Artificial Sequence
  PR000210 LCDR3 Chothia
QQHYTTPPT

SEQ ID NO: 160 - protein, 9 aa, Artificial Sequence
  PR000265 LCDR3 Chothia
QQYYGSSRT

SEQ ID NO: 161 - protein, 11 aa, Artificial Sequence
  PR000483 LCDR3 Chothia
ATYTGFGSLAV

SEQ ID NO: 162 - protein, 11 aa, Artificial Sequence
  PR000628 LCDR3 Chothia
QQRSNWPPALT

SEQ ID NO: 163 - protein, 10 aa, Artificial Sequence
  PR000151 LFWR4 Chothia, PR000210 LFWR4 Chothia, PR000265 LFWR4 Chothia
FGQGTKVEIK

SEQ ID NO: 164 - protein, 10 aa, Artificial Sequence
  PR000196 LFWR4 Chothia, PR000197 LFWR4 Chothia, PR000447 LFWR4 Chothia
FGGGTKVEIK

SEQ ID NO: 165 - protein, 10 aa, Artificial Sequence
  PR000483 LFWR4 Chothia
FGGGTKLTVL

SEQ ID NO: 166 - protein, 118 aa, Artificial Sequence [sequence omitted]

SEQ ID NO: 167 - protein, 129 aa, Artificial Sequence
  PR000196 VH
EVQLLESGGGLVQRGGSLRLSCAASGFTFSSYAMTWVRQAPGKGLEWVSAISGSGGNTYYADSVRGRFTISRDNSKNTLYLQMNSLRAEDTAVYFCAKEAYHYGSGSYYDDYYYGMDVWGQGTTVTVSS

SEQ ID NO: 168 - protein, 115 aa, Artificial Sequence
  PR000197 VH
QVQLQQWGAGLLKPSETLSLTCAVYGGSFSGYYWSWIRQPPGKGLEWIGEINHSGSTDSNPSLKGRVTFSVDTSKNQFSLKLNSVTAADTAVYYCARLTGPFDYWGQGTLVTVSS

SEQ ID NO: 169 - protein, 120 aa, Artificial Sequence [sequence omitted]

SEQ ID NO: 170 - protein, 119 aa, Artificial Sequence
  PR000265 VH
EVQLVESGGGLVQPGGSLRLSCAASGFTFSSYWMSWVRQAPGKGLEWVANIKQEGSEKYYVDSVKGRFTISRDNAKNSLYLQMNSLRAEDTAVYYCARDRAVAGAFDIWGQGTMVTVSS

SEQ ID NO: 171 - protein, 115 aa, Artificial Sequence
  PR000447 VH
QVQLQQWGAGLLKPSETLSLTCAVYGGSFSGYYWSWIRQPPGKGLEWIGEIIHSGSTDSNPSLKGRVTFSVDTSKNQFSLKLNSVTAADTAVYYCARLTGPFDYWGQGTLVTVSS

SEQ ID NO: 172 - protein, 115 aa, Artificial Sequence
  PR000448 VH, PR000980 VH
QVQLQQWGAGLLKPSETLSLTCAVYGGSFSGYYWSWIRQPPGKGLEWIGEIQHSGSTDSNPSLKGRVTFSVDTSKNQFSLKLNSVTAADTAVYYCARLTGPFDYWGQGTLVTVSS

SEQ ID NO: 173 - protein, 116 aa, Artificial Sequence
  PR000483 VH
EVQLVQSGAEVKKPGESLRISCKGSGYSFSTYWISWVRQMPGKGLEWMGKIYPGDSYTNYSPSFQGQVTISADKSISTAYLQWSSLKASDTAMYYCARGYGIFDYWGQGTLVTVSS

SEQ ID NO: 174 - protein, 121 aa, Artificial Sequence [sequence omitted]

SEQ ID NO: 175 - protein, 124 aa, Artificial Sequence
  PR001758 VH
EVQLLESGGGLVQLGGSLRLSCAASGFTFSRYAMTWVRQAPEKGLEWVSSISGSGDDTYYGDSVKGRFTISRDNSQNTVYLQMNSLRAEDTAVYFCAKEKAGTTGDYYYNVDVWGQGTTVTVSS

SEQ ID NO: 176 - protein, 124 aa, Artificial Sequence
  PR001759 VH
EVQLLESGGGLVQPGGSLRLSCAASGFTFSSYAMSWFRQPPETGLQWVSSIGGSGGDTYYADSVKGRFTISRDNSKNTLYLQMNSLRAEDTAVYYCAKEGSNGTDDNYYDVDVWGQGTTVTVSS

SEQ ID NO: 177 - protein, 124 aa, Artificial Sequence
  PR001760 VH
EVQLVESGGGVVQPGGSLRLSCAASGFTFSNYAMTWVRQAPEKGLEWVSSISGSGVSTYYADSVKGRFTISRDNSKNTLYLQMTRLTAEDTAVYFCAKEGSSETDDHYYNVDVWGQGTTVTVSS

SEQ ID NO: 178 - protein, 124 aa, Artificial Sequence
  PR001763 VH
EVQLLESGGGLVQPGGSLRLSCTASGFTFSNYAMSWVRQAPEKGLEWVSSISGSGGSTFYADSVKGRFTISRDNSKNTLYLQMNRLTAEDTAVYYCAKEGSNGTDDYHYDIDVWGQGTTVTVSS

SEQ ID NO: 179 - protein, 124 aa, Artificial Sequence
  PR001764 VH
EVQLLESGGGLVQPGGSLRLSCAASGFTFSSYAMSWVRQAPEKGLEWVSAISGGGGSTYYADSVKGRFTISRDNSKNTLYLQMDSLKAEDTAVYYCAKEGTTETDDYHYNMDVWGQGTTVTVSS

SEQ ID NO: 180 - protein, 124 aa, Artificial Sequence
  PR001766 VH
EVQLLESGGGLVQPGGSLRLSCAASGFTFSSYAMSWGRQAPGKGLEWVSSISGSGGSTYYADSVKGRFTISRDNSKNTLYLQMNSLRAEDTAVYYCAKEKTGTTGDYYYDMDVWGQGTTVTVSS

SEQ ID NO: 181 - protein, 126 aa, Artificial Sequence
  PR001767 VH
EVQLVETGGGLIQPGGSLRLSCAASGFTVSSNYMSWVRQAPGKGLEWVSVIYSDGSTYYADSVKGRFTISRDNSKNTLYLQMNSLRAEDTAVYYCARDRYYGSGNYPTAYYGMDVRGQGTTVTVSS

SEQ ID NO: 182 - protein, 124 aa, Artificial Sequence
  PR001768 VH
EVQLLESGGGLVQPGGSLRLSCAASGFTFSNYAMTWVRQAPGKGLEWVSSISGSGDSTYYADSVKGRFTISRDNSKNTLYLQMNSLRAEDTAVYYCAKEGTGTTSDYYYNVDVWGQGTTVTVSS

SEQ ID NO: 183 - protein, 124 aa, Artificial Sequence
  PR001771 VH
EVQLLESGGGLVQPGGSLRLSCAASGFTFSNYAMTWVRQPPGKGLEWVSSISGSGGSTYYADSVKGRFTISRDNSKNTLYLQMNSLRAEDTAVYYCAKEGTGTTSDYYYNVDVWGQGTTVTVSS

SEQ ID NO: 184 - protein, 124 aa, Artificial Sequence
  PR001774 VH
EVQLVESGGGLVQPGGSLRLSCAASGFTFSSFAMTWVRQAPEKGLEWVSTISGSGDTTYYADSVKGRFTISRDSSKNTLYLQMNSLRAEDSAVYFCAKEATAMASDYYYGVDVWGQGTTVTVSS

SEQ ID NO: 185 - protein, 123 aa, Artificial Sequence
  PR001775 VH
EVQLLESGGGLVQSGGSLRLSCAASGFTFSSYAMSWVRQAPGKGLEWVSAISGSGGSTDYADSVKGRFTISRDNSTNTLYLQMNSLRAEDTAVYYCAKERAYDYSNYVDFDYWGQGTLVTVSS

SEQ ID NO: 186 - protein, 125 aa, Artificial Sequence
  PR001776 VH
EVQLLESGGGLVQPGGSLRLSCAASGFTFSSYAMSWVRQAPEKGLEWVSAISSSGGSTYYADSVKGRFTISRDNSKNTLYLQMNSLRAEDTAVYYCAKDGVTTPSYYYYYDMDVWGQGTTVTVSS

SEQ ID NO: 187 - protein, 124 aa, Artificial Sequence
  PR001780 VH
EVQLLESGGGLIQPGGSLRLSCAASGFTFSSFAMTWVRQAPGKGLEWVSTISGSGDNTYYADSVKGRFTISRDNSKNTLYLQMNSLRAEDTAVYFCAKEDTAVASDYYYNIDVWGQGTTVTVSS

SEQ ID NO: 188 - protein, 124 aa, Artificial Sequence
  PR001781 VH
EVQLLESGGGLVQLGGSLRLSCAASGFTFSSYAMTWVRQAPEKGLEWVSSISGSGGNTYYADSVKGRFTISRDNSKNTLYLQMNSLRAEDTAVYYCAKERTGTTGDYYYNVDVWGQGTTVTVSS

SEQ ID NO: 189 - protein, 124 aa, Artificial Sequence
  PR001830 VH
EVQLLESGGGLVQPGGSLRLSCTASGFTFSNYAMSWVRQAPEKGLEWVSSISGSGGSTFYADSVKGRFTISRDNSKNTLYLQMNSLRAEDTAVYFCAKEGSSETDDHYYNVDVWGQGTTVTVSS

SEQ ID NO: 190 - protein, 124 aa, Artificial Sequence
  PR001831 VH
EVQLVESGGGVIQPGGSLRLSCEASGFTFSSYAMSWVRQAPEKGLEWVSSISGSGDSTYYADSVKGRFTISRDNSKNTLYLQMNSLRAEDTAGYHCAKEGSNGTDDYHYDIDVWGQGTSVTVSS

SEQ ID NO: 191 - protein, 124 aa, Artificial Sequence
  PR001833 VH
EVQLLESGGGLVQPGGSLRLSCAASGFTFSSYAMSWVRQAPEKGLEWVSSISGSGGSTFYADSVKGRFTISRDNSKNTLYLQMNSLRAEDTAVYFCAKEGATETDDYHFNTDVWGQGTTVTVSS

SEQ ID NO: 192 - protein, 124 aa, Artificial Sequence
  PR001834 VH
EVQLLESGGGLVQPGGSLRLSCAASGFTFSGYAMTWVRQPPEKGLEWVSSISGSGNNTFYADSVKGRFTISRDNSKNTLYLQMNSLRAEDTAVYYCAKEGTTETDDYHYNMDVWGQGTTVTVSS

SEQ ID NO: 193 - protein, 124 aa, Artificial Sequence
  PR001836 VH
EVQLLESGGGLVQPGGSLRLSCAASGFIFSNFAMTWVRQPPEKGLKWVSSINGSGFNTYYTDSVKGRFTISRDNSRNTLYLQMNRLTAEDTAVYFCAKEGSSETDDHYYNVDVWGQGTTVTVSS

SEQ ID NO: 194 - protein, 124 aa, Artificial Sequence
  PR001837 VH
EVQLLESGGGLVQPGGSLRLSCEASGFTFSSYAMSWVRQAPEKGLEWVSSISGSGGSTFYADSVKGRFTISRDNSKNTLYLQMNSLRAEDTAVYYCAKEGTTETDDYHYNMDVWGQGTTVTVSS

SEQ ID NO: 195 - protein, 124 aa, Artificial Sequence
  PR001838 VH
EVQLLESGGGLVQPGGSLRLSCAASGFTFSNYAMSWFRQPPETGLKWVSSIDGSGGDTYYADSVKGRFTISRDNSKNTLYLQMNSLRAEDTAVYYCAKEGSHGTDDSHYDVDVWGQGTTVTVSS

SEQ ID NO: 196 - protein, 123 aa, Artificial Sequence
  PR001840 VH
EVQLVESGGGLVQPGGSLRLSCAASGFTFSSYWMHWVRQAPGKGLVWVSRINSDGSSTSYADSVQGRFTISRDNAKNTLYLQMNSLRAEDTAVYYCVRKGSSSYYHYSIEDDWGQGTLVTVSS

SEQ ID NO: 197 - protein, 124 aa, Artificial Sequence
  PR001842 VH
EVQLLESGGGLVQPGGSLRLSCAASGFTFSSYAMSWGRQAPGKGLEWVSAISGSGGSTYYADSVKGRFTISRDNSKNTLYLHMNSLRAEDTAVYYCAKEKVATTGDYYYDMDVWGQGTTVTVSS

SEQ ID NO: 198 - protein, 124 aa, Artificial Sequence
  PR004469 VH
EVQLLESGGGLVQPGGSLRLSCAASGFTFSNYAMSWFRQPPETGLKWVSSIDASGGDTYYADSVKGRFTISRDNSKNTLYLQMNSLRAEDTAVYYCAKEGSHGTDDSHYDVDVWGQGTTVTVSS

SEQ ID NO: 199 - protein, 107 aa, Artificial Sequence [sequence omitted]

SEQ ID NO: 200 - protein, 112 aa, Artificial Sequence
  PR000196 VL
DIVMTQSPLSLPVTPGEPASISCRSSQSLLHSNGYNYLDWYLQKPGQSPQLLIFLGSNRASGVPDRFSGSGSGTDFTLKISRVEAEDVGVYYCMQALQTPLTFGGGTKVEIK

SEQ ID NO: 201 - protein, 107 aa, Artificial Sequence
  PR000197 VL
EFVMTQSPATLSVSPGERATLSCRASQSISSILAWYQQKPGQAPRLLIYGASTRATGIPARFSGSGSGTEFTLTISSLQSEDFAVYYCQQYYNWPLTFGGGTKVEIK

SEQ ID NO: 202 - protein, 107 aa, Artificial Sequence [sequence omitted]

SEQ ID NO: 203 - protein, 107 aa, Artificial Sequence
  PR000265 VL
DIQMTQSPSTLSASVGDRVTVTCRASQSIYIWLAWYQQKPGKAPNLLIYKASSLETGVPSRFSGSGSGTEFTLTISSLQPDDFATYYCQQYYGSSRTFGQGTKVEIK

SEQ ID NO: 204 - protein, 107 aa, Artificial Sequence
  PR000447 VL, PR000448 VL, PR000980 VL
EIVMTQSPATLSVSPGERATLSCRASQSISSILAWYQQKPGQAPRLLIYGASTRATGIPARFSGSGSGTEFTLTISSLQSEDFAVYYCQQYYNWPLTFGGGTKVEIK

SEQ ID NO: 205 - protein, 108 aa, Artificial Sequence
  PR000483 VL
SYELTQPPSVSVSPGQTASITCSGDNIGDQYAHWYQQKPGQSPVLVIYQDKNRPSGIPERFSGSNSGNTATLTISGTQAMDEADYYCATYTGFGSLAVFGGGTKLTVL

SEQ ID NO: 206 - protein, 109 aa, Artificial Sequence [sequence omitted]

SEQ ID NO: 207 - protein, 448 aa, Artificial Sequence
  PR000151 HC
EVQLVESGGGLVQPGGSLRLSCAASGFTFSDSWIHWVRQAPGKGLEWVAWISPYGGSTYYADSVKGRFTISADTSKNTAYLQMNSLRAEDTAVYYCARRHWPGGFDYWGQGTLVTVSSASTKGPSVFPLAPSSKSTSGGTAALGCLVKDYFPEPVTVSWNSGALTSGVHTFPAVLQSSGLYSLSSVVTVPSSSLGTQTYICNVNHKPSNTKVDKKVEPKSCDKTHTCPPCPAPELLGGPSVFLFPPKPKDTLMISRTPEVTCVVVDVSHEDPEVKFNWYVDGVEVHNAKTKPREEQYASTYRVVSVLTVLHQDWLNGKEYKCKVSNKALPAPIEKTISKAKGQPREPQVYTLPPSREEMTKNQVSLTCLVKGFYPSDIAVEWESNGQPENNYKTTPPVLDSDGSFFLYSKLTVDKSRWQQGNVFSCSVMHEALHNHYTQKSLSLSPGK

SEQ ID NO: 208 - protein, 456 aa, Artificial Sequence
  PR000196 HC
EVQLLESGGGLVQRGGSLRLSCAASGFTFSSYAMTWVRQAPGKGLEWVSAISGSGGNTYYADSVRGRFTISRDNSKNTLYLQMNSLRAEDTAVYFCAKEAYHYGSGSYYDDYYYGMDVWGQGTTVTVSSASTKGPSVFPLAPCSRSTSESTAALGCLVKDYFPEPVTVSWNSGALTSGVHTFPAVLQSSGLYSLSSVVTVPSSSLGTKTYTCNVDHKPSNTKVDKRVESKYGPPCPPCPAPEFLGGPSVFLFPPKPKDTLMISRTPEVTCVVVDVSQEDPEVQFNWYVDGVEVHNAKTKPREEQFNSTYRVVSVLTVLHQDWLNGKEYKCKVSNKGLPSSIEKTISKAKGQPREPQVYTLPPSQEEMTKNQVSLTCLVKGFYPSDIAVEWESNGQPENNYKTTPPVLDSDGSFFLYSRLTVDKSRWQEGNVFSCSVMHEALHNHYTQKSLSLSLGK

SEQ ID NO: 209 - protein, 442 aa, Artificial Sequence
  PR000197 HC
QVQLQQWGAGLLKPSETLSLTCAVYGGSFSGYYWSWIRQPPGKGLEWIGEINHSGSTDSNPSLKGRVTFSVDTSKNQFSLKLNSVTAADTAVYYCARLTGPFDYWGQGTLVTVSSASTKGPSVFPLAPCSRSTSESTAALGCLVKDYFPEPVTVSWNSGALTSGVHTFPAVLQSSGLYSLSSVVTVPSSSLGTKTYTCNVDHKPSNTKVDKRVESKYGPPCPPCPAPEFLGGPSVFLFPPKPKDTLMISRTPEVTCVVVDVSQEDPEVQFNWYVDGVEVHNAKTKPREEQFNSTYRVVSVLTVLHQDWLNGKEYKCKVSNKGLPSSIEKTISKAKGQPREPQVYTLPPSQEEMTKNQVSLTCLVKGFYPSDIAVEWESNGQPENNYKTTPPVLDSDGSFFLYSRLTVDKSRWQEGNVFSCSVMHEALHNHYTQKSLSLSLGK

SEQ ID NO: 210 - protein, 450 aa, Artificial Sequence
  PR000210 HC
EVQLVESGGGLVQPGGSLRLSCAASGFNIKDTYIHWVRQAPGKGLEWVARIYPTNGYTRYADSVKGRFTISADTSKNTAYLQMNSLRAEDTAVYYCSRWGGDGFYAMDYWGQGTLVTVSSASTKGPSVFPLAPSSKSTSGGTAALGCLVKDYFPEPVTVSWNSGALTSGVHTFPAVLQSSGLYSLSSVVTVPSSSLGTQTYICNVNHKPSNTKVDKKVEPKSCDKTHTCPPCPAPELLGGPSVFLFPPKPKDTLMISRTPEVTCVVVDVSHEDPEVKFNWYVDGVEVHNAKTKPREEQYNSTYRVVSVLTVLHQDWLNGKEYKCKVSNKALPAPIEKTISKAKGQPREPQVYTLPPSREEMTKNQVSLTCLVKGFYPSDIAVEWESNGQPENNYKTTPPVLDSDGSFFLYSKLTVDKSRWQQGNVFSCSVMHEALHNHYTQKSLSLSPGK

SEQ ID NO: 211 - protein, 449 aa, Artificial Sequence
  PR000265 HC
EVQLVESGGGLVQPGGSLRLSCAASGFTFSSYWMSWVRQAPGKGLEWVANIKQEGSEKYYVDSVKGRFTISRDNAKNSLYLQMNSLRAEDTAVYYCARDRAVAGAFDIWGQGTMVTVSSASTKGPSVFPLAPSSKSTSGGTAALGCLVKDYFPEPVTVSWNSGALTSGVHTFPAVLQSSGLYSLSSVVTVPSSSLGTQTYICNVNHKPSNTKVDKKVEPKSCDKTHTCPPCPAPELLGGPSVFLFPPKPKDTLMISRTPEVTCVVVDVSHEDPEVKFNWYVDGVEVHNAKTKPREEQYASTYRVVSVLTVLHQDWLNGKEYKCKVSNKALPAPIEKTISKAKGQPREPQVYTLPPSREEMTKNQVSLTCLVKGFYPSDIAVEWESNGQPENNYKTTPPVLDSDGSFFLYSKLTVDKSRWQQGNVFSCSVMHEALHNHYTQKSLSLSPGK

SEQ ID NO: 212 - protein, 442 aa, Artificial Sequence
  PR000447 HC
QVQLQQWGAGLLKPSETLSLTCAVYGGSFSGYYWSWIRQPPGKGLEWIGEIIHSGSTDSNPSLKGRVTFSVDTSKNQFSLKLNSVTAADTAVYYCARLTGPFDYWGQGTLVTVSSASTKGPSVFPLAPCSRSTSESTAALGCLVKDYFPEPVTVSWNSGALTSGVHTFPAVLQSSGLYSLSSVVTVPSSSLGTKTYTCNVDHKPSNTKVDKRVESKYGPPCPPCPAPEFLGGPSVFLFPPKPKDTLMISRTPEVTCVVVDVSQEDPEVQFNWYVDGVEVHNAKTKPREEQFNSTYRVVSVLTVLHQDWLNGKEYKCKVSNKGLPSSIEKTISKAKGQPREPQVYTLPPSQEEMTKNQVSLTCLVKGFYPSDIAVEWESNGQPENNYKTTPPVLDSDGSFFLYSRLTVDKSRWQEGNVFSCSVMHEALHNHYTQKSLSLSLGK

SEQ ID NO: 213 - protein, 442 aa, Artificial Sequence
  PR000448 HC
QVQLQQWGAGLLKPSETLSLTCAVYGGSFSGYYWSWIRQPPGKGLEWIGEIQHSGSTDSNPSLKGRVTFSVDTSKNQFSLKLNSVTAADTAVYYCARLTGPFDYWGQGTLVTVSSASTKGPSVFPLAPCSRSTSESTAALGCLVKDYFPEPVTVSWNSGALTSGVHTFPAVLQSSGLYSLSSVVTVPSSSLGTKTYTCNVDHKPSNTKVDKRVESKYGPPCPPCPAPEFLGGPSVFLFPPKPKDTLMISRTPEVTCVVVDVSQEDPEVQFNWYVDGVEVHNAKTKPREEQFNSTYRVVSVLTVLHQDWLNGKEYKCKVSNKGLPSSIEKTISKAKGQPREPQVYTLPPSQEEMTKNQVSLTCLVKGFYPSDIAVEWESNGQPENNYKTTPPVLDSDGSFFLYSRLTVDKSRWQEGNVFSCSVMHEALHNHYTQKSLSLSLGK

SEQ ID NO: 214 - protein, 442 aa, Artificial Sequence
  PR000483 HC
EVQLVQSGAEVKKPGESLRISCKGSGYSFSTYWISWVRQMPGKGLEWMGKIYPGDSYTNYSPSFQGQVTISADKSISTAYLQWSSLKASDTAMYYCARGYGIFDYWGQGTLVTVSSASTKGPSVFPLAPCSRSTSESTAALGCLVKDYFPEPVTVSWNSGALTSGVHTFPAVLQSSGLYSLSSVVTVPSSNFGTQTYTCNVDHKPSNTKVDKTVERKCCVECPPCPAPPVAGPSVFLFPPKPKDTLMISRTPEVTCVVVDVSHEDPEVQFNWYVDGVEVHNAKTKPREEQFNSTFRVVSVLTVVHQDWLNGKEYKCKVSNKGLPAPIEKTISKTKGQPREPQVYTLPPSREEMTKNQVSLTCLVKGFYPSDIAVEWESNGQPENNYKTTPPMLDSDGSFFLYSKLTVDKSRWQQGNVFSCSVMHEALHNHYTQKSLSLSPGK

SEQ ID NO: 215 - protein, 448 aa, Artificial Sequence
  PR000628 HC
QVQLQQWGAGLLKPSETLSLTCAVYGGSFSGYYWSWIRQSPEKGLEWIGEINHGGYVTYNPSLESRVTISVDTSKNQFSLKLSSVTAADTAVYYCARDYGPGNYDWYFDLWGRGTLVTVSSASTKGPSVFPLAPCSRSTSESTAALGCLVKDYFPEPVTVSWNSGALTSGVHTFPAVLQSSGLYSLSSVVTVPSSSLGTKTYTCNVDHKPSNTKVDKRVESKYGPPCPPCPAPEFLGGPSVFLFPPKPKDTLMISRTPEVTCVVVDVSQEDPEVQFNWYVDGVEVHNAKTKPREEQFNSTYRVVSVLTVLHQDWLNGKEYKCKVSNKGLPSSIEKTISKAKGQPREPQVYTLPPSQEEMTKNQVSLTCLVKGFYPSDIAVEWESNGQPENNYKTTPPVLDSDGSFFLYSRLTVDKSRWQEGNVFSCSVMHEALHNHYTQKSLSLSLGK

SEQ ID NO: 216 - protein, 445 aa, Artificial Sequence
  PR000980 HC
QVQLQQWGAGLLKPSETLSLTCAVYGGSFSGYYWSWIRQPPGKGLEWIGEIQHSGSTDSNPSLKGRVTFSVDTSKNQFSLKLNSVTAADTAVYYCARLTGPFDYWGQGTLVTVSSASTKGPSVFPLAPSSKSTSGGTAALGCLVKDYFPEPVTVSWNSGALTSGVHTFPAVLQSSGLYSLSSVVTVPSSSLGTQTYICNVNHKPSNTKVDKKVEPKSCDKTHTCPPCPAPEAAGGPSVFLFPPKPKDTLMISRTPEVTCVVVDVSHEDPEVKFNWYVDGVEVHNAKTKPREEQYNSTYRVVSVLTVLHQDWLNGKEYKCKVSNKALPAPIEKTISKAKGQPRRPQVYTLPPSREEMTKNQVSLTCLVKGFYPSDIAVEWESNGQPENNYKTTPPVLDSDGSFFLYSKLTVDKSRWQQGNVFSCSVMHEALHNHYTQKSLSLSPGK

SEQ ID NO: 217 - protein, 356 aa, Artificial Sequence
  PR001758 HC
EVQLLESGGGLVQLGGSLRLSCAASGFTFSRYAMTWVRQAPEKGLEWVSSISGSGDDTYYGDSVKGRFTISRDNSQNTVYLQMNSLRAEDTAVYFCAKEKAGTTGDYYYNVDVWGQGTTVTVSSEPKSCDKTHTCPPCPAPELLGGPSVFLFPPKPKDTLMISRTPEVTCVVVDVSHEDPEVKFNWYVDGVEVHNAKTKPREEQYNSTYRVVSVLTVLHQDWLNGKEYKCKVSNKALPAPIEKTISKAKGQPREPQVYTLPPSREEMTKNQVSLTCLVKGFYPSDIAVEWESNGQPENNYKTTPPVLDSDGSFFLYSKLTVDKSRWQQGNVFSCSVMHEALHNHYTQKSLSLSPGK

SEQ ID NO: 218 - protein, 356 aa, Artificial Sequence
  PR001759 HC
EVQLLESGGGLVQPGGSLRLSCAASGFTFSSYAMSWFRQPPETGLQWVSSIGGSGGDTYYADSVKGRFTISRDNSKNTLYLQMNSLRAEDTAVYYCAKEGSNGTDDNYYDVDVWGQGTTVTVSSEPKSCDKTHTCPPCPAPELLGGPSVFLFPPKPKDTLMISRTPEVTCVVVDVSHEDPEVKFNWYVDGVEVHNAKTKPREEQYNSTYRVVSVLTVLHQDWLNGKEYKCKVSNKALPAPIEKTISKAKGQPREPQVYTLPPSREEMTKNQVSLTCLVKGFYPSDIAVEWESNGQPENNYKTTPPVLDSDGSFFLYSKLTVDKSRWQQGNVFSCSVMHEALHNHYTQKSLSLSPGK

SEQ ID NO: 219 - protein, 356 aa, Artificial Sequence
  PR001760 HC
EVQLVESGGGVVQPGGSLRLSCAASGFTFSNYAMTWVRQAPEKGLEWVSSISGSGVSTYYADSVKGRFTISRDNSKNTLYLQMTRLTAEDTAVYFCAKEGSSETDDHYYNVDVWGQGTTVTVSSEPKSCDKTHTCPPCPAPELLGGPSVFLFPPKPKDTLMISRTPEVTCVVVDVSHEDPEVKFNWYVDGVEVHNAKTKPREEQYNSTYRVVSVLTVLHQDWLNGKEYKCKVSNKALPAPIEKTISKAKGQPREPQVYTLPPSREEMTKNQVSLTCLVKGFYPSDIAVEWESNGQPENNYKTTPPVLDSDGSFFLYSKLTVDKSRWQQGNVFSCSVMHEALHNHYTQKSLSLSPGK

SEQ ID NO: 220 - protein, 356 aa, Artificial Sequence
  PR001763 HC
EVQLLESGGGLVQPGGSLRLSCTASGFTFSNYAMSWVRQAPEKGLEWVSSISGSGGSTFYADSVKGRFTISRDNSKNTLYLQMNRLTAEDTAVYYCAKEGSNGTDDYHYDIDVWGQGTTVTVSSEPKSCDKTHTCPPCPAPELLGGPSVFLFPPKPKDTLMISRTPEVTCVVVDVSHEDPEVKFNWYVDGVEVHNAKTKPREEQYNSTYRVVSVLTVLHQDWLNGKEYKCKVSNKALPAPIEKTISKAKGQPREPQVYTLPPSREEMTKNQVSLTCLVKGFYPSDIAVEWESNGQPENNYKTTPPVLDSDGSFFLYSKLTVDKSRWQQGNVFSCSVMHEALHNHYTQKSLSLSPGK

SEQ ID NO: 221 - protein, 356 aa, Artificial Sequence
  PR001764 HC
EVQLLESGGGLVQPGGSLRLSCAASGFTFSSYAMSWVRQAPEKGLEWVSAISGGGGSTYYADSVKGRFTISRDNSKNTLYLQMDSLKAEDTAVYYCAKEGTTETDDYHYNMDVWGQGTTVTVSSEPKSCDKTHTCPPCPAPELLGGPSVFLFPPKPKDTLMISRTPEVTCVVVDVSHEDPEVKFNWYVDGVEVHNAKTKPREEQYNSTYRVVSVLTVLHQDWLNGKEYKCKVSNKALPAPIEKTISKAKGQPREPQVYTLPPSREEMTKNQVSLTCLVKGFYPSDIAVEWESNGQPENNYKTTPPVLDSDGSFFLYSKLTVDKSRWQQGNVFSCSVMHEALHNHYTQKSLSLSPGK

SEQ ID NO: 222 - protein, 356 aa, Artificial Sequence
  PR001766 HC
EVQLLESGGGLVQPGGSLRLSCAASGFTFSSYAMSWGRQAPGKGLEWVSSISGSGGSTYYADSVKGRFTISRDNSKNTLYLQMNSLRAEDTAVYYCAKEKTGTTGDYYYDMDVWGQGTTVTVSSEPKSCDKTHTCPPCPAPELLGGPSVFLFPPKPKDTLMISRTPEVTCVVVDVSHEDPEVKFNWYVDGVEVHNAKTKPREEQYNSTYRVVSVLTVLHQDWLNGKEYKCKVSNKALPAPIEKTISKAKGQPREPQVYTLPPSREEMTKNQVSLTCLVKGFYPSDIAVEWESNGQPENNYKTTPPVLDSDGSFFLYSKLTVDKSRWQQGNVFSCSVMHEALHNHYTQKSLSLSPGK

SEQ ID NO: 223 - protein, 358 aa, Artificial Sequence
  PR001767 HC
EVQLVETGGGLIQPGGSLRLSCAASGFTVSSNYMSWVRQAPGKGLEWVSVIYSDGSTYYADSVKGRFTISRDNSKNTLYLQMNSLRAEDTAVYYCARDRYYGSGNYPTAYYGMDVRGQGTTVTVSSEPKSCDKTHTCPPCPAPELLGGPSVFLFPPKPKDTLMISRTPEVTCVVVDVSHEDPEVKFNWYVDGVEVHNAKTKPREEQYNSTYRVVSVLTVLHQDWLNGKEYKCKVSNKALPAPIEKTISKAKGQPREPQVYTLPPSREEMTKNQVSLTCLVKGFYPSDIAVEWESNGQPENNYKTTPPVLDSDGSFFLYSKLTVDKSRWQQGNVFSCSVMHEALHNHYTQKSLSLSPGK

SEQ ID NO: 224 - protein, 356 aa, Artificial Sequence
  PR001768 HC
EVQLLESGGGLVQPGGSLRLSCAASGFTFSNYAMTWVRQAPGKGLEWVSSISGSGDSTYYADSVKGRFTISRDNSKNTLYLQMNSLRAEDTAVYYCAKEGTGTTSDYYYNVDVWGQGTTVTVSSEPKSCDKTHTCPPCPAPELLGGPSVFLFPPKPKDTLMISRTPEVTCVVVDVSHEDPEVKFNWYVDGVEVHNAKTKPREEQYNSTYRVVSVLTVLHQDWLNGKEYKCKVSNKALPAPIEKTISKAKGQPREPQVYTLPPSREEMTKNQVSLTCLVKGFYPSDIAVEWESNGQPENNYKTTPPVLDSDGSFFLYSKLTVDKSRWQQGNVFSCSVMHEALHNHYTQKSLSLSPGK

SEQ ID NO: 225 - protein, 356 aa, Artificial Sequence
  PR001771 HC
EVQLLESGGGLVQPGGSLRLSCAASGFTFSNYAMTWVRQPPGKGLEWVSSISGSGGSTYYADSVKGRFTISRDNSKNTLYLQMNSLRAEDTAVYYCAKEGTGTTSDYYYNVDVWGQGTTVTVSSEPKSCDKTHTCPPCPAPELLGGPSVFLFPPKPKDTLMISRTPEVTCVVVDVSHEDPEVKFNWYVDGVEVHNAKTKPREEQYNSTYRVVSVLTVLHQDWLNGKEYKCKVSNKALPAPIEKTISKAKGQPREPQVYTLPPSREEMTKNQVSLTCLVKGFYPSDIAVEWESNGQPENNYKTTPPVLDSDGSFFLYSKLTVDKSRWQQGNVFSCSVMHEALHNHYTQKSLSLSPGK

SEQ ID NO: 226 - protein, 356 aa, Artificial Sequence
  PR001774 HC
EVQLVESGGGLVQPGGSLRLSCAASGFTFSSFAMTWVRQAPEKGLEWVSTISGSGDTTYYADSVKGRFTISRDSSKNTLYLQMNSLRAEDSAVYFCAKEATAMASDYYYGVDVWGQGTTVTVSSEPKSCDKTHTCPPCPAPELLGGPSVFLFPPKPKDTLMISRTPEVTCVVVDVSHEDPEVKFNWYVDGVEVHNAKTKPREEQYNSTYRVVSVLTVLHQDWLNGKEYKCKVSNKALPAPIEKTISKAKGQPREPQVYTLPPSREEMTKNQVSLTCLVKGFYPSDIAVEWESNGQPENNYKTTPPVLDSDGSFFLYSKLTVDKSRWQQGNVFSCSVMHEALHNHYTQKSLSLSPGK

SEQ ID NO: 227 - protein, 355 aa, Artificial Sequence
  PR001775 HC
EVQLLESGGGLVQSGGSLRLSCAASGFTFSSYAMSWVRQAPGKGLEWVSAISGSGGSTDYADSVKGRFTISRDNSTNTLYLQMNSLRAEDTAVYYCAKERAYDYSNYVDFDYWGQGTLVTVSSEPKSCDKTHTCPPCPAPELLGGPSVFLFPPKPKDTLMISRTPEVTCVVVDVSHEDPEVKFNWYVDGVEVHNAKTKPREEQYNSTYRVVSVLTVLHQDWLNGKEYKCKVSNKALPAPIEKTISKAKGQPREPQVYTLPPSREEMTKNQVSLTCLVKGFYPSDIAVEWESNGQPENNYKTTPPVLDSDGSFFLYSKLTVDKSRWQQGNVFSCSVMHEALHNHYTQKSLSLSPGK

SEQ ID NO: 228 - protein, 357 aa, Artificial Sequence
  PR001776 HC
EVQLLESGGGLVQPGGSLRLSCAASGFTFSSYAMSWVRQAPEKGLEWVSAISSSGGSTYYADSVKGRFTISRDNSKNTLYLQMNSLRAEDTAVYYCAKDGVTTPSYYYYYDMDVWGQGTTVTVSSEPKSCDKTHTCPPCPAPELLGGPSVFLFPPKPKDTLMISRTPEVTCVVVDVSHEDPEVKFNWYVDGVEVHNAKTKPREEQYNSTYRVVSVLTVLHQDWLNGKEYKCKVSNKALPAPIEKTISKAKGQPREPQVYTLPPSREEMTKNQVSLTCLVKGFYPSDIAVEWESNGQPENNYKTTPPVLDSDGSFFLYSKLTVDKSRWQQGNVFSCSVMHEALHNHYTQKSLSLSPGK

SEQ ID NO: 229 - protein, 356 aa, Artificial Sequence
  PR001780 HC
EVQLLESGGGLIQPGGSLRLSCAASGFTFSSFAMTWVRQAPGKGLEWVSTISGSGDNTYYADSVKGRFTISRDNSKNTLYLQMNSLRAEDTAVYFCAKEDTAVASDYYYNIDVWGQGTTVTVSSEPKSCDKTHTCPPCPAPELLGGPSVFLFPPKPKDTLMISRTPEVTCVVVDVSHEDPEVKFNWYVDGVEVHNAKTKPREEQYNSTYRVVSVLTVLHQDWLNGKEYKCKVSNKALPAPIEKTISKAKGQPREPQVYTLPPSREEMTKNQVSLTCLVKGFYPSDIAVEWESNGQPENNYKTTPPVLDSDGSFFLYSKLTVDKSRWQQGNVFSCSVMHEALHNHYTQKSLSLSPGK

SEQ ID NO: 230 - protein, 356 aa, Artificial Sequence
  PR001781 HC
EVQLLESGGGLVQLGGSLRLSCAASGFTFSSYAMTWVRQAPEKGLEWVSSISGSGGNTYYADSVKGRFTISRDNSKNTLYLQMNSLRAEDTAVYYCAKERTGTTGDYYYNVDVWGQGTTVTVSSEPKSCDKTHTCPPCPAPELLGGPSVFLFPPKPKDTLMISRTPEVTCVVVDVSHEDPEVKFNWYVDGVEVHNAKTKPREEQYNSTYRVVSVLTVLHQDWLNGKEYKCKVSNKALPAPIEKTISKAKGQPREPQVYTLPPSREEMTKNQVSLTCLVKGFYPSDIAVEWESNGQPENNYKTTPPVLDSDGSFFLYSKLTVDKSRWQQGNVFSCSVMHEALHNHYTQKSLSLSPGK

SEQ ID NO: 231 - protein, 356 aa, Artificial Sequence
  PR001830 HC
EVQLLESGGGLVQPGGSLRLSCTASGFTFSNYAMSWVRQAPEKGLEWVSSISGSGGSTFYADSVKGRFTISRDNSKNTLYLQMNSLRAEDTAVYFCAKEGSSETDDHYYNVDVWGQGTTVTVSSEPKSCDKTHTCPPCPAPELLGGPSVFLFPPKPKDTLMISRTPEVTCVVVDVSHEDPEVKFNWYVDGVEVHNAKTKPREEQYNSTYRVVSVLTVLHQDWLNGKEYKCKVSNKALPAPIEKTISKAKGQPREPQVYTLPPSREEMTKNQVSLTCLVKGFYPSDIAVEWESNGQPENNYKTTPPVLDSDGSFFLYSKLTVDKSRWQQGNVFSCSVMHEALHNHYTQKSLSLSPGK

SEQ ID NO: 232 - protein, 356 aa, Artificial Sequence
  PR001831 HC
EVQLVESGGGVIQPGGSLRLSCEASGFTFSSYAMSWVRQAPEKGLEWVSSISGSGDSTYYADSVKGRFTISRDNSKNTLYLQMNSLRAEDTAGYHCAKEGSNGTDDYHYDIDVWGQGTSVTVSSEPKSCDKTHTCPPCPAPELLGGPSVFLFPPKPKDTLMISRTPEVTCVVVDVSHEDPEVKFNWYVDGVEVHNAKTKPREEQYNSTYRVVSVLTVLHQDWLNGKEYKCKVSNKALPAPIEKTISKAKGQPREPQVYTLPPSREEMTKNQVSLTCLVKGFYPSDIAVEWESNGQPENNYKTTPPVLDSDGSFFLYSKLTVDKSRWQQGNVFSCSVMHEALHNHYTQKSLSLSPGK

SEQ ID NO: 233 - protein, 356 aa, Artificial Sequence
  PR001833 HC
EVQLLESGGGLVQPGGSLRLSCAASGFTFSSYAMSWVRQAPEKGLEWVSSISGSGGSTFYADSVKGRFTISRDNSKNTLYLQMNSLRAEDTAVYFCAKEGATETDDYHFNTDVWGQGTTVTVSSEPKSCDKTHTCPPCPAPELLGGPSVFLFPPKPKDTLMISRTPEVTCVVVDVSHEDPEVKFNWYVDGVEVHNAKTKPREEQYNSTYRVVSVLTVLHQDWLNGKEYKCKVSNKALPAPIEKTISKAKGQPREPQVYTLPPSREEMTKNQVSLTCLVKGFYPSDIAVEWESNGQPENNYKTTPPVLDSDGSFFLYSKLTVDKSRWQQGNVFSCSVMHEALHNHYTQKSLSLSPGK

SEQ ID NO: 234 - protein, 356 aa, Artificial Sequence
  PR001834 HC
EVQLLESGGGLVQPGGSLRLSCAASGFTFSGYAMTWVRQPPEKGLEWVSSISGSGNNTFYADSVKGRFTISRDNSKNTLYLQMNSLRAEDTAVYYCAKEGTTETDDYHYNMDVWGQGTTVTVSSEPKSCDKTHTCPPCPAPELLGGPSVFLFPPKPKDTLMISRTPEVTCVVVDVSHEDPEVKFNWYVDGVEVHNAKTKPREEQYNSTYRVVSVLTVLHQDWLNGKEYKCKVSNKALPAPIEKTISKAKGQPREPQVYTLPPSREEMTKNQVSLTCLVKGFYPSDIAVEWESNGQPENNYKTTPPVLDSDGSFFLYSKLTVDKSRWQQGNVFSCSVMHEALHNHYTQKSLSLSPGK

SEQ ID NO: 235 - protein, 356 aa, Artificial Sequence
  PR001836 HC
EVQLLESGGGLVQPGGSLRLSCAASGFIFSNFAMTWVRQPPEKGLKWVSSINGSGFNTYYTDSVKGRFTISRDNSRNTLYLQMNRLTAEDTAVYFCAKEGSSETDDHYYNVDVWGQGTTVTVSSEPKSCDKTHTCPPCPAPELLGGPSVFLFPPKPKDTLMISRTPEVTCVVVDVSHEDPEVKFNWYVDGVEVHNAKTKPREEQYNSTYRVVSVLTVLHQDWLNGKEYKCKVSNKALPAPIEKTISKAKGQPREPQVYTLPPSREEMTKNQVSLTCLVKGFYPSDIAVEWESNGQPENNYKTTPPVLDSDGSFFLYSKLTVDKSRWQQGNVFSCSVMHEALHNHYTQKSLSLSPGK

SEQ ID NO: 236 - protein, 356 aa, Artificial Sequence
  PR001837 HC
EVQLLESGGGLVQPGGSLRLSCEASGFTFSSYAMSWVRQAPEKGLEWVSSISGSGGSTFYADSVKGRFTISRDNSKNTLYLQMNSLRAEDTAVYYCAKEGTTETDDYHYNMDVWGQGTTVTVSSEPKSCDKTHTCPPCPAPELLGGPSVFLFPPKPKDTLMISRTPEVTCVVVDVSHEDPEVKFNWYVDGVEVHNAKTKPREEQYNSTYRVVSVLTVLHQDWLNGKEYKCKVSNKALPAPIEKTISKAKGQPREPQVYTLPPSREEMTKNQVSLTCLVKGFYPSDIAVEWESNGQPENNYKTTPPVLDSDGSFFLYSKLTVDKSRWQQGNVFSCSVMHEALHNHYTQKSLSLSPGK

SEQ ID NO: 237 - protein, 356 aa, Artificial Sequence
  PR001838 HC
EVQLLESGGGLVQPGGSLRLSCAASGFTFSNYAMSWFRQPPETGLKWVSSIDGSGGDTYYADSVKGRFTISRDNSKNTLYLQMNSLRAEDTAVYYCAKEGSHGTDDSHYDVDVWGQGTTVTVSSEPKSCDKTHTCPPCPAPELLGGPSVFLFPPKPKDTLMISRTPEVTCVVVDVSHEDPEVKFNWYVDGVEVHNAKTKPREEQYNSTYRVVSVLTVLHQDWLNGKEYKCKVSNKALPAPIEKTISKAKGQPREPQVYTLPPSREEMTKNQVSLTCLVKGFYPSDIAVEWESNGQPENNYKTTPPVLDSDGSFFLYSKLTVDKSRWQQGNVFSCSVMHEALHNHYTQKSLSLSPGK

SEQ ID NO: 238 - protein, 355 aa, Artificial Sequence
  PR001840 HC
EVQLVESGGGLVQPGGSLRLSCAASGFTFSSYWMHWVRQAPGKGLVWVSRINSDGSSTSYADSVQGRFTISRDNAKNTLYLQMNSLRAEDTAVYYCVRKGSSSYYHYSIEDDWGQGTLVTVSSEPKSCDKTHTCPPCPAPELLGGPSVFLFPPKPKDTLMISRTPEVTCVVVDVSHEDPEVKFNWYVDGVEVHNAKTKPREEQYNSTYRVVSVLTVLHQDWLNGKEYKCKVSNKALPAPIEKTISKAKGQPREPQVYTLPPSREEMTKNQVSLTCLVKGFYPSDIAVEWESNGQPENNYKTTPPVLDSDGSFFLYSKLTVDKSRWQQGNVFSCSVMHEALHNHYTQKSLSLSPGK

SEQ ID NO: 239 - protein, 356 aa, Artificial Sequence
  PR001842 HC
EVQLLESGGGLVQPGGSLRLSCAASGFTFSSYAMSWGRQAPGKGLEWVSAISGSGGSTYYADSVKGRFTISRDNSKNTLYLHMNSLRAEDTAVYYCAKEKVATTGDYYYDMDVWGQGTTVTVSSEPKSCDKTHTCPPCPAPELLGGPSVFLFPPKPKDTLMISRTPEVTCVVVDVSHEDPEVKFNWYVDGVEVHNAKTKPREEQYNSTYRVVSVLTVLHQDWLNGKEYKCKVSNKALPAPIEKTISKAKGQPREPQVYTLPPSREEMTKNQVSLTCLVKGFYPSDIAVEWESNGQPENNYKTTPPVLDSDGSFFLYSKLTVDKSRWQQGNVFSCSVMHEALHNHYTQKSLSLSPGK

SEQ ID NO: 240 - protein, 356 aa, Artificial Sequence
  PR004469 HC
EVQLLESGGGLVQPGGSLRLSCAASGFTFSNYAMSWFRQPPETGLKWVSSIDASGGDTYYADSVKGRFTISRDNSKNTLYLQMNSLRAEDTAVYYCAKEGSHGTDDSHYDVDVWGQGTTVTVSSEPKSCDKTHTCPPCPAPELLGGPSVFLFPPKPKDTLMISRTPEVTCVVVDVSHEDPEVKFNWYVDGVEVHNAKTKPREEQYNSTYRVVSVLTVLHQDWLNGKEYKCKVSNKALPAPIEKTISKAKGQPREPQVYTLPPSREEMTKNQVSLTCLVKGFYPSDIAVEWESNGQPENNYKTTPPVLDSDGSFFLYSKLTVDKSRWQQGNVFSCSVMHEALHNHYTQKSLSLSPGK

SEQ ID NO: 241 - protein, 214 aa, Artificial Sequence
  PR000151 LC
DIQMTQSPSSLSASVGDRVTITCRASQDVSTAVAWYQQKPGKAPKLLIYSASFLYSGVPSRFSGSGSGTDFTLTISSLQPEDFATYYCQQYLYHPATFGQGTKVEIKRTVAAPSVFIFPPSDEQLKSGTASVVCLLNNFYPREAKVQWKVDNALQSGNSQESVTEQDSKDSTYSLSSTLTLSKADYEKHKVYACEVTHQGLSSPVTKSFNRGEC

SEQ ID NO: 242 - protein, 219 aa, Artificial Sequence
  PR000196 LC
DIVMTQSPLSLPVTPGEPASISCRSSQSLLHSNGYNYLDWYLQKPGQSPQLLIFLGSNRASGVPDRFSGSGSGTDFTLKISRVEAEDVGVYYCMQALQTPLTFGGGTKVEIKRTVAAPSVFIFPPSDEQLKSGTASVVCLLNNFYPREAKVQWKVDNALQSGNSQESVTEQDSKDSTYSLSSTLTLSKADYEKHKVYACEVTHQGLSSPVTKSFNRGEC

SEQ ID NO: 243 - protein, 214 aa, Artificial Sequence
  PR000197 LC
EFVMTQSPATLSVSPGERATLSCRASQSISSILAWYQQKPGQAPRLLIYGASTRATGIPARFSGSGSGTEFTLTISSLQSEDFAVYYCQQYYNWPLTFGGGTKVEIKRTVAAPSVFIFPPSDEQLKSGTASVVCLLNNFYPREAKVQWKVDNALQSGNSQESVTEQDSKDSTYSLSSTLTLSKADYEKHKVYACEVTHQGLSSPVTKSFNRGEC

SEQ ID NO: 244 - protein, 214 aa, Artificial Sequence
  PR000210 LC, PR001212 Chain, PR002811 Chain, PR002812 Chain, PR002813
DIQMTQSPSSLSASVGDRVTITCRASQDVNTAVAWYQQKPGKAPKLLIYSASFLYSGVPSRFSGSRSGTDFTLTISSLQPEDFATYYCQQHYTTPPTFGQGTKVEIKRTVAAPSVFIFPPSDEQLKSGTASVVCLLNNFYPREAKVQWKVDNALQSGNSQESVTEQDSKDSTYSLSSTLTLSKADYEKHKVYACEVTHQGLSSPVTKSFNRGEC

SEQ ID NO: 245 - protein, 214 aa, Artificial Sequence
  PR000265 LC, PR003549 Chain, PR003550 Chain, PR003551 Chain, PR004268
DIQMTQSPSTLSASVGDRVTVTCRASQSIYIWLAWYQQKPGKAPNLLIYKASSLETGVPSRFSGSGSGTEFTLTISSLQPDDFATYYCQQYYGSSRTFGQGTKVEIKRTVAAPSVFIFPPSDEQLKSGTASVVCLLNNFYPREAKVQWKVDNALQSGNSQESVTEQDSKDSTYSLSSTLTLSKADYEKHKVYACEVTHQGLSSPVTKSFNRGEC

SEQ ID NO: 246 - protein, 214 aa, Artificial Sequence
  PR000447 LC, PR000448 LC, PR000701 Chain, PR000980 LC, PR003052 Chain
EIVMTQSPATLSVSPGERATLSCRASQSISSILAWYQQKPGQAPRLLIYGASTRATGIPARFSGSGSGTEFTLTISSLQSEDFAVYYCQQYYNWPLTFGGGTKVEIKRTVAAPSVFIFPPSDEQLKSGTASVVCLLNNFYPREAKVQWKVDNALQSGNSQESVTEQDSKDSTYSLSSTLTLSKADYEKHKVYACEVTHQGLSSPVTKSFNRGEC

SEQ ID NO: 247 - protein, 214 aa, Artificial Sequence
  PR000483 LC
SYELTQPPSVSVSPGQTASITCSGDNIGDQYAHWYQQKPGQSPVLVIYQDKNRPSGIPERFSGSNSGNTATLTISGTQAMDEADYYCATYTGFGSLAVFGGGTKLTVLGQPKAAPSVTLFPPSSEELQANKATLVCLISDFYPGAVTVAWKADSSPVKAGVETTTPSKQSNNKYAASSYLSLTPEQWKSHRSYSCQVTHEGSTVEKTVAPTECS

SEQ ID NO: 248 - protein, 216 aa, Artificial Sequence
  PR000628 LC
EIVLTQSPATLSLSPGERATLSCRASQSVSSYLAWYQQKPGQAPRLLIYDASNRATGIPARFSGSGSGTDFTLTISSLEPEDFAVYYCQQRSNWPPALTFGGGTKVEIKRTVAAPSVFIFPPSDEQLKSGTASVVCLLNNFYPREAKVQWKVDNALQSGNSQESVTEQDSKDSTYSLSSTLTLSKADYEKHKVYACEVTHQGLSSPVTKSFNRGEC

SEQ ID NO: 249 - protein, 222 aa, Artificial Sequence
  PR000701 Chain, PR004270 Chain
EVQLVESGGGLVQPGGSLRLSCAASGFTFSSYWMSWVRQAPGKGLEWVANIKQEGSEKYYVDSVKGRFTISRDNAKNSLYLQMNSLRAEDTAVYYCARDRAVAGAFDIWGQGTMVTVSSASTKGPSVFPLAPSSKSTSGGTAALGCLVKDYFPEPVTVSWNSGALTSGVHTFPAVLQSSGLYSLSSVVTVPSSSLGTQTYICNVNHKPSNTKVDKKVEPKSC

SEQ ID NO: 250 - protein, 656 aa, Artificial Sequence
  PR000701 Chain
DIQMTQSPSTLSASVGDRVTVTCRASQSIYIWLAWYQQKPGKAPNLLIYKASSLETGVPSRFSGSGSGTEFTLTISSLQPDDFATYYCQQYYGSSRTFGQGTKVEIKRTVAAPSVFIFPPSDEQLKSGTASVVCLLNNFYPREAKVQWKVDNALQSGNSQESVTEQDSKDSTYSLSSTLTLSKADYEKHKVYACEVTHQGLSSPVTKSFNRGECQVQLQQWGAGLLKPSETLSLTCAVYGGSFSGYYWSWIRQPPGKGLEWIGEINHSGSTDSNPSLKGRVTFSVDTSKNQFSLKLNSVTAADTAVYYCARLTGPFDYWGQGTLVTVSSASTKGPSVFPLAPCSRSTSESTAALGCLVKDYFPEPVTVSWNSGALTSGVHTFPAVLQSSGLYSLSSVVTVPSSSLGTKTYTCNVDHKPSNTKVDKRVESKYGPPCPPCPAPEFLGGPSVFLFPPKPKDTLMISRTPEVTCVVVDVSQEDPEVQFNWYVDGVEVHNAKTKPREEQFNSTYRVVSVLTVLHQDWLNGKEYKCKVSNKGLPSSIEKTISKAKGQPREPQVYTLPPSQEEMTKNQVSLTCLVKGFYPSDIAVEWESNGQPENNYKTTPPVLDSDGSFFLYSRLTVDKSRWQEGNVFSCSVMHEALHNHYTQKSLSLSLGK

SEQ ID NO: 251 - protein, 705 aa, Artificial Sequence
  PR001212 Chain
EVQLVESGGGLVQPGGSLRLSCAASGFNIKDTYIHWVRQAPGKGLEWVARIYPTNGYTRYADSVKGRFTISADTSKNTAYLQMNSLRAEDTAVYYCSRWGGDGFYAMDYWGQGTLVTVSSASTKGPSVFPLAPSSKSTSGGTAALGCLVKDYFPEPVTVSWNSGALTSGVHTFPAVLQSSGLYSLSSVVTVPSSSLGTQTYICNVNHKPSNTKVDKKVEPKSCDKTHTCPPCPAPELLGGPSVFLFPPKPKDTLMISRTPEVTCVVVDVSHEDPEVKFNWYVDGVEVHNAKTKPREEQYNSTYRVVSVLTVLHQDWLNGKEYKCKVSNKALPAPIEKTISKAKGQPREPQVYTLPPSREEMTKNQVSLTCLVKGFYPSDIAVEWESNGQPENNYKTTPPVLDSDGSFFLYSKLTVDKSRWQQGNVFSCSVMHEALHNHYTQKSLSLSPGKLEPKSSDKTHTPPPPPRTQVQLQQWGAGLLKPSETLSLTCAVYGGSFSGYYWSWIRQPPGKGLEWIGEIQHSGSTDSNPSLKGRVTFSVDTSKNQFSLKLNSVTAADTAVYYCARLTGPFDYWGQGTLVTVSSGGGGSGGGGSGGGGSEIVMTQSPATLSVSPGERATLSCRASQSISSILAWYQQKPGQAPRLLIYGASTRATGIPARFSGSGSGTEFTLTISSLQSEDFAVYYCQQYYNWPLTFGGGTKVEIK

SEQ ID NO: 252 - protein, 703 aa, Artificial Sequence
  PR002811 Chain
EVQLVESGGGLVQPGGSLRLSCAASGFNIKDTYIHWVRQAPGKGLEWVARIYPTNGYTRYADSVKGRFTISADTSKNTAYLQMNSLRAEDTAVYYCSRWGGDGFYAMDYWGQGTLVTVSSASTKGPSVFPLAPSSKSTSGGTAALGCLVKDYFPEPVTVSWNSGALTSGVHTFPAVLQSSGLYSLSSVVTVPSSSLGTQTYICNVNHKPSNTKVDKKVEPKSCDKTHTCPPCPAPEAAGGPSVFLFPPKPKDTLMISRTPEVTCVVVDVSHEDPEVKFNWYVDGVEVHNAKTKPREEQYNSTYRVVSVLTVLHQDWLNGKEYKCKVSNKALGAPIEKTISKAKGQPREPQVYTLPPSREEMTKNQVSLTCLVKGFYPSDIAVEWESNGQPENNYKTTPPVLDSDGSFFLYSKLTVDKSRWQQGNVFSCSVMHEALHNHYTQKSLSLSPGEPKSSDKTHTPPPPPRTQVQLQQWGAGLLKPSETLSLTCAVYGGSFSGYYWSWIRQPPGKGLEWIGEIQHSGSTDSNPSLKGRVTFSVDTSKNQFSLKLNSVTAADTAVYYCARLTGPFDYWGQGTLVTVSSGGGGSGGGGSGGGGSEIVMTQSPATLSVSPGERATLSCRASQSISSILAWYQQKPGQAPRLLIYGASTRATGIPARFSGSGSGTEFTLTISSLQSEDFAVYYCQQYYNWPLTFGGGTKVEIK

SEQ ID NO: 253 - protein, 590 aa, Artificial Sequence
  PR002812 Chain
EVQLVESGGGLVQPGGSLRLSCAASGFNIKDTYIHWVRQAPGKGLEWVARIYPTNGYTRYADSVKGRFTISADTSKNTAYLQMNSLRAEDTAVYYCSRWGGDGFYAMDYWGQGTLVTVSSASTKGPSVFPLAPSSKSTSGGTAALGCLVKDYFPEPVTVSWNSGALTSGVHTFPAVLQSSGLYSLSSVVTVPSSSLGTQTYICNVNHKPSNTKVDKKVEPKSCDKTHTCPPCPAPEAAGGPSVFLFPPKPKDTLMISRTPEVTCVVVDVSHEDPEVKFNWYVDGVEVHNAKTKPREEQYNSTYRVVSVLTVLHQDWLNGKEYKCKVSNKALGAPIEKTISKAKGQPREPQVYTLPPSREEMTKNQVSLTCLVKGFYPSDIAVEWESNGQPENNYKTTPPVLDSDGSFFLYSKLTVDKSRWQQGNVFSCSVMHEALHNHYTQKSLSLSPGEPKSSDKTHTPPPPPRTEVQLLESGGGLVQLGGSLRLSCAASGFTFSRYAMTWVRQAPEKGLEWVSSISGSGDDTYYGDSVKGRFTISRDNSQNTVYLQMNSLRAEDTAVYFCAKEKAGTTGDYYYNVDVWGQGTTVTVSS

SEQ ID NO: 254 - protein, 590 aa, Artificial Sequence
  PR002813 Chain
EVQLVESGGGLVQPGGSLRLSCAASGFNIKDTYIHWVRQAPGKGLEWVARIYPTNGYTRYADSVKGRFTISADTSKNTAYLQMNSLRAEDTAVYYCSRWGGDGFYAMDYWGQGTLVTVSSASTKGPSVFPLAPSSKSTSGGTAALGCLVKDYFPEPVTVSWNSGALTSGVHTFPAVLQSSGLYSLSSVVTVPSSSLGTQTYICNVNHKPSNTKVDKKVEPKSCDKTHTCPPCPAPEAAGGPSVFLFPPKPKDTLMISRTPEVTCVVVDVSHEDPEVKFNWYVDGVEVHNAKTKPREEQYNSTYRVVSVLTVLHQDWLNGKEYKCKVSNKALGAPIEKTISKAKGQPREPQVYTLPPSREEMTKNQVSLTCLVKGFYPSDIAVEWESNGQPENNYKTTPPVLDSDGSFFLYSKLTVDKSRWQQGNVFSCSVMHEALHNHYTQKSLSLSPGEPKSSDKTHTPPPPPRTEVQLVESGGGVVQPGGSLRLSCAASGFTFSNYAMTWVRQAPEKGLEWVSSISGSGVSTYYADSVKGRFTISRDNSKNTLYLQMTRLTAEDTAVYFCAKEGSSETDDHYYNVDVWGQGTTVTVSS

SEQ ID NO: 255 - protein, 590 aa, Artificial Sequence
  PR002815 Chain
EVQLVESGGGLVQPGGSLRLSCAASGFNIKDTYIHWVRQAPGKGLEWVARIYPTNGYTRYADSVKGRFTISADTSKNTAYLQMNSLRAEDTAVYYCSRWGGDGFYAMDYWGQGTLVTVSSASTKGPSVFPLAPSSKSTSGGTAALGCLVKDYFPEPVTVSWNSGALTSGVHTFPAVLQSSGLYSLSSVVTVPSSSLGTQTYICNVNHKPSNTKVDKKVEPKSCDKTHTCPPCPAPEAAGGPSVFLFPPKPKDTLMISRTPEVTCVVVDVSHEDPEVKFNWYVDGVEVHNAKTKPREEQYNSTYRVVSVLTVLHQDWLNGKEYKCKVSNKALGAPIEKTISKAKGQPREPQVYTLPPSREEMTKNQVSLTCLVKGFYPSDIAVEWESNGQPENNYKTTPPVLDSDGSFFLYSKLTVDKSRWQQGNVFSCSVMHEALHNHYTQKSLSLSPGEPKSSDKTHTPPPPPRTEVQLLESGGGLVQPGGSLRLSCAASGFTFSSYAMSWVRQAPEKGLEWVSAISGGGGSTYYADSVKGRFTISRDNSKNTLYLQMDSLKAEDTAVYYCAKEGTTETDDYHYNMDVWGQGTTVTVSS

SEQ ID NO: 256 - protein, 590 aa, Artificial Sequence
  PR002820 Chain
EVQLVESGGGLVQPGGSLRLSCAASGFNIKDTYIHWVRQAPGKGLEWVARIYPTNGYTRYADSVKGRFTISADTSKNTAYLQMNSLRAEDTAVYYCSRWGGDGFYAMDYWGQGTLVTVSSASTKGPSVFPLAPSSKSTSGGTAALGCLVKDYFPEPVTVSWNSGALTSGVHTFPAVLQSSGLYSLSSVVTVPSSSLGTQTYICNVNHKPSNTKVDKKVEPKSCDKTHTCPPCPAPEAAGGPSVFLFPPKPKDTLMISRTPEVTCVVVDVSHEDPEVKFNWYVDGVEVHNAKTKPREEQYNSTYRVVSVLTVLHQDWLNGKEYKCKVSNKALGAPIEKTISKAKGQPREPQVYTLPPSREEMTKNQVSLTCLVKGFYPSDIAVEWESNGQPENNYKTTPPVLDSDGSFFLYSKLTVDKSRWQQGNVFSCSVMHEALHNHYTQKSLSLSPGEPKSSDKTHTPPPPPRTEVQLVESGGGLVQPGGSLRLSCAASGFTFSSFAMTWVRQAPEKGLEWVSTISGSGDTTYYADSVKGRFTISRDSSKNTLYLQMNSLRAEDSAVYFCAKEATAMASDYYYGVDVWGQGTTVTVSS

SEQ ID NO: 257 - protein, 589 aa, Artificial Sequence
  PR002821 Chain
EVQLVESGGGLVQPGGSLRLSCAASGFNIKDTYIHWVRQAPGKGLEWVARIYPTNGYTRYADSVKGRFTISADTSKNTAYLQMNSLRAEDTAVYYCSRWGGDGFYAMDYWGQGTLVTVSSASTKGPSVFPLAPSSKSTSGGTAALGCLVKDYFPEPVTVSWNSGALTSGVHTFPAVLQSSGLYSLSSVVTVPSSSLGTQTYICNVNHKPSNTKVDKKVEPKSCDKTHTCPPCPAPEAAGGPSVFLFPPKPKDTLMISRTPEVTCVVVDVSHEDPEVKFNWYVDGVEVHNAKTKPREEQYNSTYRVVSVLTVLHQDWLNGKEYKCKVSNKALGAPIEKTISKAKGQPREPQVYTLPPSREEMTKNQVSLTCLVKGFYPSDIAVEWESNGQPENNYKTTPPVLDSDGSFFLYSKLTVDKSRWQQGNVFSCSVMHEALHNHYTQKSLSLSPGEPKSSDKTHTPPPPPRTEVQLLESGGGLVQSGGSLRLSCAASGFTFSSYAMSWVRQAPGKGLEWVSAISGSGGSTDYADSVKGRFTISRDNSTNTLYLQMNSLRAEDTAVYYCAKERAYDYSNYVDFDYWGQGTLVTVSS

SEQ ID NO: 258 - protein, 590 aa, Artificial Sequence
  PR002822 Chain
EVQLVESGGGLVQPGGSLRLSCAASGFNIKDTYIHWVRQAPGKGLEWVARIYPTNGYTRYADSVKGRFTISADTSKNTAYLQMNSLRAEDTAVYYCSRWGGDGFYAMDYWGQGTLVTVSSASTKGPSVFPLAPSSKSTSGGTAALGCLVKDYFPEPVTVSWNSGALTSGVHTFPAVLQSSGLYSLSSVVTVPSSSLGTQTYICNVNHKPSNTKVDKKVEPKSCDKTHTCPPCPAPEAAGGPSVFLFPPKPKDTLMISRTPEVTCVVVDVSHEDPEVKFNWYVDGVEVHNAKTKPREEQYNSTYRVVSVLTVLHQDWLNGKEYKCKVSNKALGAPIEKTISKAKGQPREPQVYTLPPSREEMTKNQVSLTCLVKGFYPSDIAVEWESNGQPENNYKTTPPVLDSDGSFFLYSKLTVDKSRWQQGNVFSCSVMHEALHNHYTQKSLSLSPGEPKSSDKTHTPPPPPRTEVQLLESGGGLIQPGGSLRLSCAASGFTFSSFAMTWVRQAPGKGLEWVSTISGSGDNTYYADSVKGRFTISRDNSKNTLYLQMNSLRAEDTAVYFCAKEDTAVASDYYYNIDVWGQGTTVTVSS

SEQ ID NO: 259 - protein, 590 aa, Artificial Sequence
  PR002823 Chain
EVQLVESGGGLVQPGGSLRLSCAASGFNIKDTYIHWVRQAPGKGLEWVARIYPTNGYTRYADSVKGRFTISADTSKNTAYLQMNSLRAEDTAVYYCSRWGGDGFYAMDYWGQGTLVTVSSASTKGPSVFPLAPSSKSTSGGTAALGCLVKDYFPEPVTVSWNSGALTSGVHTFPAVLQSSGLYSLSSVVTVPSSSLGTQTYICNVNHKPSNTKVDKKVEPKSCDKTHTCPPCPAPEAAGGPSVFLFPPKPKDTLMISRTPEVTCVVVDVSHEDPEVKFNWYVDGVEVHNAKTKPREEQYNSTYRVVSVLTVLHQDWLNGKEYKCKVSNKALGAPIEKTISKAKGQPREPQVYTLPPSREEMTKNQVSLTCLVKGFYPSDIAVEWESNGQPENNYKTTPPVLDSDGSFFLYSKLTVDKSRWQQGNVFSCSVMHEALHNHYTQKSLSLSPGEPKSSDKTHTPPPPPRTEVQLLESGGGLVQLGGSLRLSCAASGFTFSSYAMTWVRQAPEKGLEWVSSISGSGGNTYYADSVKGRFTISRDNSKNTLYLQMNSLRAEDTAVYYCAKERTGTTGDYYYNVDVWGQGTTVTVSS

SEQ ID NO: 260 - protein, 590 aa, Artificial Sequence
  PR002824 Chain
EVQLVESGGGLVQPGGSLRLSCAASGFNIKDTYIHWVRQAPGKGLEWVARIYPTNGYTRYADSVKGRFTISADTSKNTAYLQMNSLRAEDTAVYYCSRWGGDGFYAMDYWGQGTLVTVSSASTKGPSVFPLAPSSKSTSGGTAALGCLVKDYFPEPVTVSWNSGALTSGVHTFPAVLQSSGLYSLSSVVTVPSSSLGTQTYICNVNHKPSNTKVDKKVEPKSCDKTHTCPPCPAPEAAGGPSVFLFPPKPKDTLMISRTPEVTCVVVDVSHEDPEVKFNWYVDGVEVHNAKTKPREEQYNSTYRVVSVLTVLHQDWLNGKEYKCKVSNKALGAPIEKTISKAKGQPREPQVYTLPPSREEMTKNQVSLTCLVKGFYPSDIAVEWESNGQPENNYKTTPPVLDSDGSFFLYSKLTVDKSRWQQGNVFSCSVMHEALHNHYTQKSLSLSPGEPKSSDKTHTPPPPPRTEVQLLESGGGLVQPGGSLRLSCTASGFTFSNYAMSWVRQAPEKGLEWVSSISGSGGSTFYADSVKGRFTISRDNSKNTLYLQMNSLRAEDTAVYFCAKEGSSETDDHYYNVDVWGQGTTVTVSS

SEQ ID NO: 261 - protein, 590 aa, Artificial Sequence
  PR002825 Chain
EVQLVESGGGLVQPGGSLRLSCAASGFNIKDTYIHWVRQAPGKGLEWVARIYPTNGYTRYADSVKGRFTISADTSKNTAYLQMNSLRAEDTAVYYCSRWGGDGFYAMDYWGQGTLVTVSSASTKGPSVFPLAPSSKSTSGGTAALGCLVKDYFPEPVTVSWNSGALTSGVHTFPAVLQSSGLYSLSSVVTVPSSSLGTQTYICNVNHKPSNTKVDKKVEPKSCDKTHTCPPCPAPEAAGGPSVFLFPPKPKDTLMISRTPEVTCVVVDVSHEDPEVKFNWYVDGVEVHNAKTKPREEQYNSTYRVVSVLTVLHQDWLNGKEYKCKVSNKALGAPIEKTISKAKGQPREPQVYTLPPSREEMTKNQVSLTCLVKGFYPSDIAVEWESNGQPENNYKTTPPVLDSDGSFFLYSKLTVDKSRWQQGNVFSCSVMHEALHNHYTQKSLSLSPGEPKSSDKTHTPPPPPRTEVQLVESGGGVIQPGGSLRLSCEASGFTFSSYAMSWVRQAPEKGLEWVSSISGSGDSTYYADSVKGRFTISRDNSKNTLYLQMNSLRAEDTAGYHCAKEGSNGTDDYHYDIDVWGQGTSVTVSS

SEQ ID NO: 262 - protein, 590 aa, Artificial Sequence
  PR002826 Chain
EVQLVESGGGLVQPGGSLRLSCAASGFNIKDTYIHWVRQAPGKGLEWVARIYPTNGYTRYADSVKGRFTISADTSKNTAYLQMNSLRAEDTAVYYCSRWGGDGFYAMDYWGQGTLVTVSSASTKGPSVFPLAPSSKSTSGGTAALGCLVKDYFPEPVTVSWNSGALTSGVHTFPAVLQSSGLYSLSSVVTVPSSSLGTQTYICNVNHKPSNTKVDKKVEPKSCDKTHTCPPCPAPEAAGGPSVFLFPPKPKDTLMISRTPEVTCVVVDVSHEDPEVKFNWYVDGVEVHNAKTKPREEQYNSTYRVVSVLTVLHQDWLNGKEYKCKVSNKALGAPIEKTISKAKGQPREPQVYTLPPSREEMTKNQVSLTCLVKGFYPSDIAVEWESNGQPENNYKTTPPVLDSDGSFFLYSKLTVDKSRWQQGNVFSCSVMHEALHNHYTQKSLSLSPGEPKSSDKTHTPPPPPRTEVQLLESGGGLVQPGGSLRLSCAASGFTFSSYAMSWVRQAPEKGLEWVSSISGSGGSTFYADSVKGRFTISRDNSKNTLYLQMNSLRAEDTAVYFCAKEGATETDDYHFNTDVWGQGTTVTVSS

SEQ ID NO: 263 - protein, 590 aa, Artificial Sequence
  PR002827 Chain
EVQLVESGGGLVQPGGSLRLSCAASGFNIKDTYIHWVRQAPGKGLEWVARIYPTNGYTRYADSVKGRFTISADTSKNTAYLQMNSLRAEDTAVYYCSRWGGDGFYAMDYWGQGTLVTVSSASTKGPSVFPLAPSSKSTSGGTAALGCLVKDYFPEPVTVSWNSGALTSGVHTFPAVLQSSGLYSLSSVVTVPSSSLGTQTYICNVNHKPSNTKVDKKVEPKSCDKTHTCPPCPAPEAAGGPSVFLFPPKPKDTLMISRTPEVTCVVVDVSHEDPEVKFNWYVDGVEVHNAKTKPREEQYNSTYRVVSVLTVLHQDWLNGKEYKCKVSNKALGAPIEKTISKAKGQPREPQVYTLPPSREEMTKNQVSLTCLVKGFYPSDIAVEWESNGQPENNYKTTPPVLDSDGSFFLYSKLTVDKSRWQQGNVFSCSVMHEALHNHYTQKSLSLSPGEPKSSDKTHTPPPPPRTEVQLLESGGGLVQPGGSLRLSCAASGFIFSNFAMTWVRQPPEKGLKWVSSINGSGFNTYYTDSVKGRFTISRDNSRNTLYLQMNRLTAEDTAVYFCAKEGSSETDDHYYNVDVWGQGTTVTVSS

SEQ ID NO: 264 - protein, 590 aa, Artificial Sequence
  PR002828 Chain
EVQLVESGGGLVQPGGSLRLSCAASGFNIKDTYIHWVRQAPGKGLEWVARIYPTNGYTRYADSVKGRFTISADTSKNTAYLQMNSLRAEDTAVYYCSRWGGDGFYAMDYWGQGTLVTVSSASTKGPSVFPLAPSSKSTSGGTAALGCLVKDYFPEPVTVSWNSGALTSGVHTFPAVLQSSGLYSLSSVVTVPSSSLGTQTYICNVNHKPSNTKVDKKVEPKSCDKTHTCPPCPAPEAAGGPSVFLFPPKPKDTLMISRTPEVTCVVVDVSHEDPEVKFNWYVDGVEVHNAKTKPREEQYNSTYRVVSVLTVLHQDWLNGKEYKCKVSNKALGAPIEKTISKAKGQPREPQVYTLPPSREEMTKNQVSLTCLVKGFYPSDIAVEWESNGQPENNYKTTPPVLDSDGSFFLYSKLTVDKSRWQQGNVFSCSVMHEALHNHYTQKSLSLSPGEPKSSDKTHTPPPPPRTEVQLLESGGGLVQPGGSLRLSCAASGFTFSNYAMSWFRQPPETGLKWVSSIDGSGGDTYYADSVKGRFTISRDNSKNTLYLQMNSLRAEDTAVYYCAKEGSHGTDDSHYDVDVWGQGTTVTVSS

SEQ ID NO: 265 - protein, 589 aa, Artificial Sequence
  PR002829 Chain
EVQLVESGGGLVQPGGSLRLSCAASGFNIKDTYIHWVRQAPGKGLEWVARIYPTNGYTRYADSVKGRFTISADTSKNTAYLQMNSLRAEDTAVYYCSRWGGDGFYAMDYWGQGTLVTVSSASTKGPSVFPLAPSSKSTSGGTAALGCLVKDYFPEPVTVSWNSGALTSGVHTFPAVLQSSGLYSLSSVVTVPSSSLGTQTYICNVNHKPSNTKVDKKVEPKSCDKTHTCPPCPAPEAAGGPSVFLFPPKPKDTLMISRTPEVTCVVVDVSHEDPEVKFNWYVDGVEVHNAKTKPREEQYNSTYRVVSVLTVLHQDWLNGKEYKCKVSNKALGAPIEKTISKAKGQPREPQVYTLPPSREEMTKNQVSLTCLVKGFYPSDIAVEWESNGQPENNYKTTPPVLDSDGSFFLYSKLTVDKSRWQQGNVFSCSVMHEALHNHYTQKSLSLSPGEPKSSDKTHTPPPPPRTEVQLVESGGGLVQPGGSLRLSCAASGFTFSSYWMHWVRQAPGKGLVWVSRINSDGSSTSYADSVQGRFTISRDNAKNTLYLQMNSLRAEDTAVYYCVRKGSSSYYHYSIEDDWGQGTLVTVSS

SEQ ID NO: 266 - protein, 221 aa, Artificial Sequence
  PR003052 Chain
EVQLVESGGGLVQPGGSLRLSCAASGFTFSDSWIHWVRQAPGKGLEWVAWISPYGGSTYYADSVKGRFTISADTSKNTAYLQMNSLRAEDTAVYYCARRHWPGGFDYWGQGTLVTVSSASTKGPSVFPLAPSSKSTSGGTAALGCLVKDYFPEPVTVSWNSGALTSGVHTFPAVLQSSGLYSLSSVVTVPSSSLGTQTYICNVNHKPSNTKVDKKVEPKSC

SEQ ID NO: 267 - protein, 656 aa, Artificial Sequence
  PR003052 Chain
DIQMTQSPSSLSASVGDRVTITCRASQDVSTAVAWYQQKPGKAPKLLIYSASFLYSGVPSRFSGSGSGTDFTLTISSLQPEDFATYYCQQYLYHPATFGQGTKVEIKRTVAAPSVFIFPPSDEQLKSGTASVVCLLNNFYPREAKVQWKVDNALQSGNSQESVTEQDSKDSTYSLSSTLTLSKADYEKHKVYACEVTHQGLSSPVTKSFNRGECQVQLQQWGAGLLKPSETLSLTCAVYGGSFSGYYWSWIRQPPGKGLEWIGEIQHSGSTDSNPSLKGRVTFSVDTSKNQFSLKLNSVTAADTAVYYCARLTGPFDYWGQGTLVTVSSASTKGPSVFPLAPCSRSTSESTAALGCLVKDYFPEPVTVSWNSGALTSGVHTFPAVLQSSGLYSLSSVVTVPSSSLGTKTYTCNVDHKPSNTKVDKRVESKYGPPCPPCPAPEFLGGPSVFLFPPKPKDTLMISRTPEVTCVVVDVSQEDPEVQFNWYVDGVEVHNAKTKPREEQFNSTYRVVSVLTVLHQDWLNGKEYKCKVSNKGLPSSIEKTISKAKGQPREPQVYTLPPSQEEMTKNQVSLTCLVKGFYPSDIAVEWESNGQPENNYKTTPPVLDSDGSFFLYSRLTVDKSRWQEGNVFSCSVMHEALHNHYTQKSLSLSLGK

SEQ ID NO: 268 - protein, 589 aa, Artificial Sequence
  PR003549 Chain
EVQLVESGGGLVQPGGSLRLSCAASGFTFSSYWMSWVRQAPGKGLEWVANIKQEGSEKYYVDSVKGRFTISRDNAKNSLYLQMNSLRAEDTAVYYCARDRAVAGAFDIWGQGTMVTVSSASTKGPSVFPLAPSSKSTSGGTAALGCLVKDYFPEPVTVSWNSGALTSGVHTFPAVLQSSGLYSLSSVVTVPSSSLGTQTYICNVNHKPSNTKVDKKVEPKSCDKTHTCPPCPAPEAAGGPSVFLFPPKPKDTLMISRTPEVTCVVVDVSHEDPEVKFNWYVDGVEVHNAKTKPREEQYNSTYRVVSVLTVLHQDWLNGKEYKCKVSNKALGAPIEKTISKAKGQPREPQVYTLPPSREEMTKNQVSLTCLVKGFYPSDIAVEWESNGQPENNYKTTPPVLDSDGSFFLYSKLTVDKSRWQQGNVFSCSVMHEALHNHYTQKSLSLSPGEPKSSDKTHTPPPPPRTEVQLLESGGGLVQLGGSLRLSCAASGFTFSRYAMTWVRQAPEKGLEWVSSISGSGDDTYYGDSVKGRFTISRDNSQNTVYLQMNSLRAEDTAVYFCAKEKAGTTGDYYYNVDVWGQGTTVTVSS

SEQ ID NO: 269 - protein, 589 aa, Artificial Sequence
  PR003550 Chain
EVQLVESGGGLVQPGGSLRLSCAASGFTFSSYWMSWVRQAPGKGLEWVANIKQEGSEKYYVDSVKGRFTISRDNAKNSLYLQMNSLRAEDTAVYYCARDRAVAGAFDIWGQGTMVTVSSASTKGPSVFPLAPSSKSTSGGTAALGCLVKDYFPEPVTVSWNSGALTSGVHTFPAVLQSSGLYSLSSVVTVPSSSLGTQTYICNVNHKPSNTKVDKKVEPKSCDKTHTCPPCPAPEAAGGPSVFLFPPKPKDTLMISRTPEVTCVVVDVSHEDPEVKFNWYVDGVEVHNAKTKPREEQYNSTYRVVSVLTVLHQDWLNGKEYKCKVSNKALGAPIEKTISKAKGQPREPQVYTLPPSREEMTKNQVSLTCLVKGFYPSDIAVEWESNGQPENNYKTTPPVLDSDGSFFLYSKLTVDKSRWQQGNVFSCSVMHEALHNHYTQKSLSLSPGEPKSSDKTHTPPPPPRTEVQLVESGGGVVQPGGSLRLSCAASGFTFSNYAMTWVRQAPEKGLEWVSSISGSGVSTYYADSVKGRFTISRDNSKNTLYLQMTRLTAEDTAVYFCAKEGSSETDDHYYNVDVWGQGTTVTVSS

SEQ ID NO: 270 - protein, 589 aa, Artificial Sequence
  PR003551 Chain
EVQLVESGGGLVQPGGSLRLSCAASGFTFSSYWMSWVRQAPGKGLEWVANIKQEGSEKYYVDSVKGRFTISRDNAKNSLYLQMNSLRAEDTAVYYCARDRAVAGAFDIWGQGTMVTVSSASTKGPSVFPLAPSSKSTSGGTAALGCLVKDYFPEPVTVSWNSGALTSGVHTFPAVLQSSGLYSLSSVVTVPSSSLGTQTYICNVNHKPSNTKVDKKVEPKSCDKTHTCPPCPAPEAAGGPSVFLFPPKPKDTLMISRTPEVTCVVVDVSHEDPEVKFNWYVDGVEVHNAKTKPREEQYNSTYRVVSVLTVLHQDWLNGKEYKCKVSNKALGAPIEKTISKAKGQPREPQVYTLPPSREEMTKNQVSLTCLVKGFYPSDIAVEWESNGQPENNYKTTPPVLDSDGSFFLYSKLTVDKSRWQQGNVFSCSVMHEALHNHYTQKSLSLSPGEPKSSDKTHTPPPPPRTEVQLLESGGGLVQPGGSLRLSCAASGFIFSNFAMTWVRQPPEKGLKWVSSINGSGFNTYYTDSVKGRFTISRDNSRNTLYLQMNRLTAEDTAVYFCAKEGSSETDDHYYNVDVWGQGTTVTVSS

SEQ ID NO: 271 - protein, 588 aa, Artificial Sequence
  PR004268 Chain
EVQLVESGGGVVQPGGSLRLSCAASGFTFSNYAMTWVRQAPEKGLEWVSSISGSGVSTYYADSVKGRFTISRDNSKNTLYLQMTRLTAEDTAVYFCAKEGSSETDDHYYNVDVWGQGTTVTVSSGGGGSGGGGSGGGGSEVQLVESGGGLVQPGGSLRLSCAASGFTFSSYWMSWVRQAPGKGLEWVANIKQEGSEKYYVDSVKGRFTISRDNAKNSLYLQMNSLRAEDTAVYYCARDRAVAGAFDIWGQGTMVTVSSASTKGPSVFPLAPSSKSTSGGTAALGCLVKDYFPEPVTVSWNSGALTSGVHTFPAVLQSSGLYSLSSVVTVPSSSLGTQTYICNVNHKPSNTKVDKKVEPKSCDKTHTCPPCPAPEAAGGPSVFLFPPKPKDTLMISRTPEVTCVVVDVSHEDPEVKFNWYVDGVEVHNAKTKPREEQYNSTYRVVSVLTVLHQDWLNGKEYKCKVSNKALPAPIEKTISKAKGQPREPQVYTLPPSREEMTKNQVSLTCLVKGFYPSDIAVEWESNGQPENNYKTTPPVLDSDGSFFLYSKLTVDKSRWQQGNVFSCSVMHEALHNHYTQKSLSLSPGK

SEQ ID NO: 272 - protein, 585 aa, Artificial Sequence
  PR004270 Chain
DIQMTQSPSTLSASVGDRVTVTCRASQSIYIWLAWYQQKPGKAPNLLIYKASSLETGVPSRFSGSGSGTEFTLTISSLQPDDFATYYCQQYYGSSRTFGQGTKVEIKRTVAAPSVFIFPPSDEQLKSGTASVVCLLNNFYPREAKVQWKVDNALQSGNSQESVTEQDSKDSTYSLSSTLTLSKADYEKHKVYACEVTHQGLSSPVTKSFNRGECEPKSSDKTHTPPPPPEVQLVESGGGVVQPGGSLRLSCAASGFTFSNYAMTWVRQAPEKGLEWVSSISGSGVSTYYADSVKGRFTISRDNSKNTLYLQMTRLTAEDTAVYFCAKEGSSETDDHYYNVDVWGQGTTVTVSSEPKSSDKTHTCPPCPAPEAAGGPSVFLFPPKPKDTLMISRTPEVTCVVVDVSHEDPEVKFNWYVDGVEVHNAKTKPREEQYNSTYRVVSVLTVLHQDWLNGKEYKCKVSNKALPAPIEKTISKAKGQPREPQVYTLPPSREEMTKNQVSLTCLVKGFYPSDIAVEWESNGQPENNYKTTPPVLDSDGSFFLYSKLTVDKSRWQQGNVFSCSVMHEALHNHYTQKSLSLSPGK

SEQ ID NO: 273 - protein, 4 aa, Artificial Sequence
  GS_4
GSGS

SEQ ID NO: 274 - protein, 5 aa, Artificial Sequence
  GS_5
GGGGS

SEQ ID NO: 275 - protein, 6 aa, Artificial Sequence
  GS_6
GGSGGS

SEQ ID NO: 276 - protein, 7 aa, Artificial Sequence
  GS_7
GGGGSGS

SEQ ID NO: 277 - protein, 15 aa, Artificial Sequence
  GS_15
GGGGSGGGGSGGGGS

SEQ ID NO: 278 - protein, 20 aa, Artificial Sequence
  GS_20
GGGGSGGGGSGGGGSGGGGS

SEQ ID NO: 279 - protein, 25 aa, Artificial Sequence
  GS_25
GGGGSGGGGSGGGGSGGGGSGGGGS

SEQ ID NO: 280 - protein, 15 aa, Artificial Sequence
  human IgG1 hinge
EPKSCDKTHTCPPCP

SEQ ID NO: 281 - protein, 15 aa, Artificial Sequence
  human IgG1 hinge (C220S)
EPKSSDKTHTCPPCP

SEQ ID NO: 282 - protein, 15 aa, Artificial Sequence
  H1_15
EPKSSDKTHTPPPPP

SEQ ID NO: 283 - protein, 15 aa, Artificial Sequence
  G5-LH
GGGGGDKTHTCPPCP

SEQ ID NO: 284 - protein, 17 aa, Artificial Sequence
  H1_15-RT
EPKSSDKTHTPPPPPRT

SEQ ID NO: 285 - protein, 18 aa, Artificial Sequence
  L-GS_15-RT
LGGGGSGGGGSGGGGSRT

SEQ ID NO: 286 - protein, 18 aa, Artificial Sequence
  L-H1_15-RT
LEPKSSDKTHTPPPPPRT

SEQ ID NO: 287 - protein, 19 aa, Artificial Sequence
  KL-H1_15-RT
KLEPKSSDKTHTPPPPPRT

SEQ ID NO: 288 - protein, 19 aa, Artificial Sequence
  KL-H1_15-AS
KLEPKSSDKTHTPPPPPAS

SEQ ID NO: 289 - protein, 9 aa, Artificial Sequence
  RT-GS_5-KL
RTGGGGSKL

SEQ ID NO: 290 - protein, 19 aa, Artificial Sequence
  RT-GS_15-KL
RTGGGGSGGGGSGGGGSKL

SEQ ID NO: 291 - protein, 29 aa, Artificial Sequence
  RT-GS_25-KL
RTGGGGSGGGGSGGGGSGGGGSGGGGSKL

SEQ ID NO: 292 - protein, 6 aa, Artificial Sequence
  EPKSSD
EPKSSD

SEQ ID NO: 293 - protein, 17 aa, Artificial Sequence
  AS-GS_15
ASGGGGSGGGGSGGGGS

SEQ ID NO: 294 - protein, 25 aa, Artificial Sequence
  PR007286 HFWR1 Chothia, PR007288 HFWR1 Chothia, PR007289 HFWR1 Chothia
EVQLVESGGGLVKPGGSLRLSCAAS

SEQ ID NO: 295 - protein, 25 aa, Artificial Sequence
  PR007287 HFWR1 Chothia
EVQLEESGGGLVKPGGSLRLSCAAS

SEQ ID NO: 296 - protein, 25 aa, Artificial Sequence
  PR007290 HFWR1 Chothia
EVQLVESGGGVVQPGRSLRLSCAAS

SEQ ID NO: 297 - protein, 25 aa, Artificial Sequence
  PR007291 HFWR1 Chothia
EVQLVESGGGLVKPGGSLRLSCVTS

SEQ ID NO: 298 - protein, 25 aa, Artificial Sequence
  PR007294 HFWR1 Chothia, PR007296 HFWR1 Chothia
EVQLVESGGGLVKPGGSLRLSCVAS

SEQ ID NO: 299 - protein, 25 aa, Artificial Sequence
  PR007300 HFWR1 Chothia
EVQLVESGGGLVKPGGSLRLSCTTS

SEQ ID NO: 300 - protein, 7 aa, Artificial Sequence
  PR007286 HCDR1 Chothia, PR007287 HCDR1 Chothia, PR007288 HCDR1 Chothia
GFTFSDY

SEQ ID NO: 301 - protein, 19 aa, Artificial Sequence
  PR007286 HFWR2 Chothia, PR007292 HFWR2 Chothia, PR007295 HFWR2 Chothia
YMSWIRQAPGKGLEWVSYI

SEQ ID NO: 302 - protein, 19 aa, Artificial Sequence
  PR007287 HFWR2 Chothia, PR007288 HFWR2 Chothia, PR007289 HFWR2 Chothia
YMSWFRQAPGKGLEWVSYI

SEQ ID NO: 303 - protein, 19 aa, Artificial Sequence
  PR007291 HFWR2 Chothia
YMNWIRQAPGKGQEWVSYI

SEQ ID NO: 304 - protein, 19 aa, Artificial Sequence
  PR007298 HFWR2 Chothia
YMSWVRQAPGKGLEWVSYI

SEQ ID NO: 305 - protein, 19 aa, Artificial Sequence
  PR007299 HFWR2 Chothia
QMSWLRQAPGKGLEWVSYI

SEQ ID NO: 306 - protein, 19 aa, Artificial Sequence
  PR007300 HFWR2 Chothia
YMNWVRQAPGKGLEWVSYI

SEQ ID NO: 307 - protein, 19 aa, Artificial Sequence
  PR007381 HFWR2 Chothia
AMSWVRQAPGKGLEWVSSI

SEQ ID NO: 308 - protein, 6 aa, Artificial Sequence
  PR007286 HCDR2 Chothia, PR007289 HCDR2 Chothia, PR007292 HCDR2 Chothia
SSSGST

SEQ ID NO: 309 - protein, 6 aa, Artificial Sequence
  PR007287 HCDR2 Chothia
SSSGSI

SEQ ID NO: 310 - protein, 6 aa, Artificial Sequence
  PR007288 HCDR2 Chothia
SGSGSI

SEQ ID NO: 311 - protein, 6 aa, Artificial Sequence
  PR007290 HCDR2 Chothia
SSSGTT

SEQ ID NO: 312 - protein, 6 aa, Artificial Sequence
  PR007291 HCDR2 Chothia
SGNGST

SEQ ID NO: 313 - protein, 6 aa, Artificial Sequence
  PR007293 HCDR2 Chothia
NSSGST

SEQ ID NO: 314 - protein, 6 aa, Artificial Sequence
  PR007294 HCDR2 Chothia, PR007296 HCDR2 Chothia
SGSGTT

SEQ ID NO: 315 - protein, 6 aa, Artificial Sequence
  PR007295 HCDR2 Chothia, PR007300 HCDR2 Chothia
SNNGST

SEQ ID NO: 316 - protein, 6 aa, Artificial Sequence
  PR007297 HCDR2 Chothia
SRSGST

SEQ ID NO: 317 - protein, 6 aa, Artificial Sequence
  PR007299 HCDR2 Chothia
SSSGRT

SEQ ID NO: 318 - protein, 41 aa, Artificial Sequence
  PR007286 HFWR3 Chothia, PR007291 HFWR3 Chothia, PR007295 HFWR3 Chothia
IYYADSVKGRFTISRDNAKNSLYLQMNSLRAEDTAVYYCAR

SEQ ID NO: 319 - protein, 41 aa, Artificial Sequence
  PR007287 HFWR3 Chothia
TDYADAVKGRFNISRDNAKNSLYLQMNSLRAEDTAVYYCAR

SEQ ID NO: 320 - protein, 41 aa, Artificial Sequence
  PR007288 HFWR3 Chothia
IDYADSVKGRFTISRDNAKNSLYLQMNSLRAEDTAVYYCSR

SEQ ID NO: 321 - protein, 41 aa, Artificial Sequence
  PR007289 HFWR3 Chothia
QDYADSVKGRFTISRDNAKNSLYLQMNSLRAEDTAVYYCAR

SEQ ID NO: 322 - protein, 41 aa, Artificial Sequence
  PR007290 HFWR3 Chothia, PR007292 HFWR3 Chothia, PR007294 HFWR3 Chothia
IDYADSVKGRFTISRDNAKNSLYLQMNSLRAEDTAVYYCAR

SEQ ID NO: 323 - protein, 41 aa, Artificial Sequence
  PR007293 HFWR3 Chothia
IYYEYSVKGRFTISRDNAKNSLYLQMNSLRAEDTAVYYCAR

SEQ ID NO: 324 - protein, 41 aa, Artificial Sequence
  PR007298 HFWR3 Chothia
IDYADSVKGRFTISRDNAKNSLFLEMNSLRAEDTAVYYCAR

SEQ ID NO: 325 - protein, 41 aa, Artificial Sequence
  PR007299 HFWR3 Chothia
IYYADSVKGRFTISRDNAKNSVSLQMNSLRAEDTAVYYCAR

SEQ ID NO: 326 - protein, 13 aa, Artificial Sequence
  PR007286 HCDR3 Chothia
VKPVAGTWDWFDP

SEQ ID NO: 327 - protein, 13 aa, Artificial Sequence
  PR007287 HCDR3 Chothia, PR007296 HCDR3 Chothia
EREAVAGTLDFDN

SEQ ID NO: 328 - protein, 13 aa, Artificial Sequence
  PR007288 HCDR3 Chothia
EREAVAGTLDFDY

SEQ ID NO: 329 - protein, 13 aa, Artificial Sequence
  PR007289 HCDR3 Chothia, PR007294 HCDR3 Chothia
EREPVAGTLDFDN

SEQ ID NO: 330 - protein, 13 aa, Artificial Sequence
  PR007290 HCDR3 Chothia, PR007293 HCDR3 Chothia
EREEVAGTLDFDY

SEQ ID NO: 331 - protein, 15 aa, Artificial Sequence
  PR007291 HCDR3 Chothia, PR007295 HCDR3 Chothia, PR007297 HCDR3 Chothia
VRPGGSGNYWDWFDP

SEQ ID NO: 332 - protein, 13 aa, Artificial Sequence
  PR007292 HCDR3 Chothia
EREEVAGTLDYDN

SEQ ID NO: 333 - protein, 13 aa, Artificial Sequence
  PR007298 HCDR3 Chothia
EREEVAGTLDFDN

SEQ ID NO: 334 - protein, 5 aa, Artificial Sequence
  PR007299 HCDR3 Chothia
EGRFF

SEQ ID NO: 335 - protein, 11 aa, Artificial Sequence
  PR007286 HFWR4 Chothia, PR007289 HFWR4 Chothia, PR007290 HFWR4 Chothia
WGQGTPVTVSS

SEQ ID NO: 336 - protein, 11 aa, Artificial Sequence
  PR007299 HFWR4 Chothia
PGQGTPVTVSS

SEQ ID NO: 337 - protein, 122 aa, Artificial Sequence
  PR007286 VH
EVQLVESGGGLVKPGGSLRLSCAASGFTFSDYYMSWIRQAPGKGLEWVSYISSSGSTIYYADSVKGRFTISRDNAKNSLYLQMNSLRAEDTAVYYCARVKPVAGTWDWFDPWGQGTPVTVSS

SEQ ID NO: 338 - protein, 122 aa, Artificial Sequence
  PR007287 VH
EVQLEESGGGLVKPGGSLRLSCAASGFTFSDYYMSWFRQAPGKGLEWVSYISSSGSITDYADAVKGRFNISRDNAKNSLYLQMNSLRAEDTAVYYCAREREAVAGTLDFDNWGQGTLVTVSS

SEQ ID NO: 339 - protein, 122 aa, Artificial Sequence
  PR007288 VH
EVQLVESGGGLVKPGGSLRLSCAASGFTFSDYYMSWFRQAPGKGLEWVSYISGSGSIIDYADSVKGRFTISRDNAKNSLYLQMNSLRAEDTAVYYCSREREAVAGTLDFDYWGQGTLVTVSS

SEQ ID NO: 340 - protein, 122 aa, Artificial Sequence
  PR007289 VH
EVQLVESGGGLVKPGGSLRLSCAASGFTFSDYYMSWFRQAPGKGLEWVSYISSSGSTQDYADSVKGRFTISRDNAKNSLYLQMNSLRAEDTAVYYCAREREPVAGTLDFDNWGQGTPVTVSS

SEQ ID NO: 341 - protein, 122 aa, Artificial Sequence
  PR007290 VH
EVQLVESGGGVVQPGRSLRLSCAASGFTFSDYYMSWFRQAPGKGLEWVSYISSSGTTIDYADSVKGRFTISRDNAKNSLYLQMNSLRAEDTAVYYCAREREEVAGTLDFDYWGQGTPVTVSS

SEQ ID NO: 342 - protein, 124 aa, Artificial Sequence
  PR007291 VH
EVQLVESGGGLVKPGGSLRLSCVTSGFTFSDYYMNWIRQAPGKGQEWVSYISGNGSTIYYADSVKGRFTISRDNAKNSLYLQMNSLRAEDTAVYYCARVRPGGSGNYWDWFDPWGQGTPVTVSS

SEQ ID NO: 343 - protein, 122 aa, Artificial Sequence
  PR007292 VH
EVQLVESGGGLVKPGGSLRLSCAASGFTFSDYYMSWIRQAPGKGLEWVSYISSSGSTIDYADSVKGRFTISRDNAKNSLYLQMNSLRAEDTAVYYCAREREEVAGTLDYDNWGQGTLVTVSS

SEQ ID NO: 344 - protein, 122 aa, Artificial Sequence
  PR007293 VH
EVQLVESGGGLVKPGGSLRLSCAASGFTFSDYYMSWFRQAPGKGLEWVSYINSSGSTIYYEYSVKGRFTISRDNAKNSLYLQMNSLRAEDTAVYYCAREREEVAGTLDFDYWGQGTLVTVSS

SEQ ID NO: 345 - protein, 122 aa, Artificial Sequence
  PR007294 VH
EVQLVESGGGLVKPGGSLRLSCVASGFTFSDYYMSWFRQAPGKGLEWVSYISGSGTTIDYADSVKGRFTISRDNAKNSLYLQMNSLRAEDTAVYYCAREREPVAGTLDFDNWGQGTLVTVSS

SEQ ID NO: 346 - protein, 124 aa, Artificial Sequence
  PR007295 VH
EVQLVESGGGLVKPGGSLRLSCAASGFTFSDYYMSWIRQAPGKGLEWVSYISNNGSTIYYADSVKGRFTISRDNAKNSLYLQMNSLRAEDTAVYYCARVRPGGSGNYWDWFDPWGQGTMVTVSS

SEQ ID NO: 347 - protein, 122 aa, Artificial Sequence
  PR007296 VH
EVQLVESGGGLVKPGGSLRLSCVASGFTFSDYYMSWFRQAPGKGLEWVSYISGSGTTIDYADSVKGRFTISRDNAKNSLYLQMNSLRAEDTAVYYCAREREAVAGTLDFDNWGQGTPVTVSS

SEQ ID NO: 348 - protein, 124 aa, Artificial Sequence
  PR007297 VH
EVQLVESGGGLVKPGGSLRLSCAASGFTFSDYYMSWIRQAPGKGLEWVSYISRSGSTIYYADSVKGRFTISRDNAKNSLYLQMNSLRAEDTAVYYCARVRPGGSGNYWDWFDPWGQGTLVTVSS

SEQ ID NO: 349 - protein, 122 aa, Artificial Sequence
  PR007298 VH
EVQLVESGGGLVKPGGSLRLSCAASGFTFSDYYMSWVRQAPGKGLEWVSYISSSGSTIDYADSVKGRFTISRDNAKNSLFLEMNSLRAEDTAVYYCAREREEVAGTLDFDNWGQGTLVTVSS

SEQ ID NO: 350 - protein, 114 aa, Artificial Sequence
  PR007299 VH
EVQLVESGGGLVKPGGSLRLSCAASGFTFSDYQMSWLRQAPGKGLEWVSYISSSGRTIYYADSVKGRFTISRDNAKNSVSLQMNSLRAEDTAVYYCAREGRFFPGQGTPVTVSS

SEQ ID NO: 351 - protein, 124 aa, Artificial Sequence
  PR007300 VH
EVQLVESGGGLVKPGGSLRLSCTTSGFTFSDYYMNWVRQAPGKGLEWVSYISNNGSTIYYADSVKGRFTISRDNAKNSLYLQMNSLRAEDTAVYYCARVRPGGSGNYWDWFDPWGQGTPVTVSS

SEQ ID NO: 352 - protein, 124 aa, Artificial Sequence
  PR007381 VH
EVQLLESGGGLVQPGGSLRLSCAASGFTFSNYAMSWVRQAPGKGLEWVSSIDASGGDTYYADSVKGRFTISRDNSKNTLYLQMNSLRAEDTAVYYCAKEGSHGTDDSHYDVDVWGQGTTVTVSS

SEQ ID NO: 353 - protein, 354 aa, Artificial Sequence
  PR007286 HC
EVQLVESGGGLVKPGGSLRLSCAASGFTFSDYYMSWIRQAPGKGLEWVSYISSSGSTIYYADSVKGRFTISRDNAKNSLYLQMNSLRAEDTAVYYCARVKPVAGTWDWFDPWGQGTPVTVSSEPKSSDKTHTCPPCPAPELLGGPSVFLFPPKPKDTLMISRTPEVTCVVVDVSHEDPEVKFNWYVDGVEVHNAKTKPREEQYNSTYRVVSVLTVLHQDWLNGKEYKCKVSNKALPAPIEKTISKAKGQPREPQVYTLPPSREEMTKNQVSLTCLVKGFYPSDIAVEWESNGQPENNYKTTPPVLDSDGSFFLYSKLTVDKSRWQQGNVFSCSVMHEALHNHYTQKSLSLSPGK

SEQ ID NO: 354 - protein, 354 aa, Artificial Sequence
  PR007287 HC
EVQLEESGGGLVKPGGSLRLSCAASGFTFSDYYMSWFRQAPGKGLEWVSYISSSGSITDYADAVKGRFNISRDNAKNSLYLQMNSLRAEDTAVYYCAREREAVAGTLDFDNWGQGTLVTVSSEPKSSDKTHTCPPCPAPELLGGPSVFLFPPKPKDTLMISRTPEVTCVVVDVSHEDPEVKFNWYVDGVEVHNAKTKPREEQYNSTYRVVSVLTVLHQDWLNGKEYKCKVSNKALPAPIEKTISKAKGQPREPQVYTLPPSREEMTKNQVSLTCLVKGFYPSDIAVEWESNGQPENNYKTTPPVLDSDGSFFLYSKLTVDKSRWQQGNVFSCSVMHEALHNHYTQKSLSLSPGK

SEQ ID NO: 355 - protein, 354 aa, Artificial Sequence
  PR007288 HC
EVQLVESGGGLVKPGGSLRLSCAASGFTFSDYYMSWFRQAPGKGLEWVSYISGSGSIIDYADSVKGRFTISRDNAKNSLYLQMNSLRAEDTAVYYCSREREAVAGTLDFDYWGQGTLVTVSSEPKSSDKTHTCPPCPAPELLGGPSVFLFPPKPKDTLMISRTPEVTCVVVDVSHEDPEVKFNWYVDGVEVHNAKTKPREEQYNSTYRVVSVLTVLHQDWLNGKEYKCKVSNKALPAPIEKTISKAKGQPREPQVYTLPPSREEMTKNQVSLTCLVKGFYPSDIAVEWESNGQPENNYKTTPPVLDSDGSFFLYSKLTVDKSRWQQGNVFSCSVMHEALHNHYTQKSLSLSPGK

SEQ ID NO: 356 - protein, 354 aa, Artificial Sequence
  PR007289 HC
EVQLVESGGGLVKPGGSLRLSCAASGFTFSDYYMSWFRQAPGKGLEWVSYISSSGSTQDYADSVKGRFTISRDNAKNSLYLQMNSLRAEDTAVYYCAREREPVAGTLDFDNWGQGTPVTVSSEPKSSDKTHTCPPCPAPELLGGPSVFLFPPKPKDTLMISRTPEVTCVVVDVSHEDPEVKFNWYVDGVEVHNAKTKPREEQYNSTYRVVSVLTVLHQDWLNGKEYKCKVSNKALPAPIEKTISKAKGQPREPQVYTLPPSREEMTKNQVSLTCLVKGFYPSDIAVEWESNGQPENNYKTTPPVLDSDGSFFLYSKLTVDKSRWQQGNVFSCSVMHEALHNHYTQKSLSLSPGK

SEQ ID NO: 357 - protein, 354 aa, Artificial Sequence
  PR007290 HC
EVQLVESGGGVVQPGRSLRLSCAASGFTFSDYYMSWFRQAPGKGLEWVSYISSSGTTIDYADSVKGRFTISRDNAKNSLYLQMNSLRAEDTAVYYCAREREEVAGTLDFDYWGQGTPVTVSSEPKSSDKTHTCPPCPAPELLGGPSVFLFPPKPKDTLMISRTPEVTCVVVDVSHEDPEVKFNWYVDGVEVHNAKTKPREEQYNSTYRVVSVLTVLHQDWLNGKEYKCKVSNKALPAPIEKTISKAKGQPREPQVYTLPPSREEMTKNQVSLTCLVKGFYPSDIAVEWESNGQPENNYKTTPPVLDSDGSFFLYSKLTVDKSRWQQGNVFSCSVMHEALHNHYTQKSLSLSPGK

SEQ ID NO: 358 - protein, 356 aa, Artificial Sequence
  PR007291 HC
EVQLVESGGGLVKPGGSLRLSCVTSGFTFSDYYMNWIRQAPGKGQEWVSYISGNGSTIYYADSVKGRFTISRDNAKNSLYLQMNSLRAEDTAVYYCARVRPGGSGNYWDWFDPWGQGTPVTVSSEPKSSDKTHTCPPCPAPELLGGPSVFLFPPKPKDTLMISRTPEVTCVVVDVSHEDPEVKFNWYVDGVEVHNAKTKPREEQYNSTYRVVSVLTVLHQDWLNGKEYKCKVSNKALPAPIEKTISKAKGQPREPQVYTLPPSREEMTKNQVSLTCLVKGFYPSDIAVEWESNGQPENNYKTTPPVLDSDGSFFLYSKLTVDKSRWQQGNVFSCSVMHEALHNHYTQKSLSLSPGK

SEQ ID NO: 359 - protein, 354 aa, Artificial Sequence
  PR007292 HC
EVQLVESGGGLVKPGGSLRLSCAASGFTFSDYYMSWIRQAPGKGLEWVSYISSSGSTIDYADSVKGRFTISRDNAKNSLYLQMNSLRAEDTAVYYCAREREEVAGTLDYDNWGQGTLVTVSSEPKSSDKTHTCPPCPAPELLGGPSVFLFPPKPKDTLMISRTPEVTCVVVDVSHEDPEVKFNWYVDGVEVHNAKTKPREEQYNSTYRVVSVLTVLHQDWLNGKEYKCKVSNKALPAPIEKTISKAKGQPREPQVYTLPPSREEMTKNQVSLTCLVKGFYPSDIAVEWESNGQPENNYKTTPPVLDSDGSFFLYSKLTVDKSRWQQGNVFSCSVMHEALHNHYTQKSLSLSPGK

SEQ ID NO: 360 - protein, 354 aa, Artificial Sequence
  PR007293 HC
EVQLVESGGGLVKPGGSLRLSCAASGFTFSDYYMSWFRQAPGKGLEWVSYINSSGSTIYYEYSVKGRFTISRDNAKNSLYLQMNSLRAEDTAVYYCAREREEVAGTLDFDYWGQGTLVTVSSEPKSSDKTHTCPPCPAPELLGGPSVFLFPPKPKDTLMISRTPEVTCVVVDVSHEDPEVKFNWYVDGVEVHNAKTKPREEQYNSTYRVVSVLTVLHQDWLNGKEYKCKVSNKALPAPIEKTISKAKGQPREPQVYTLPPSREEMTKNQVSLTCLVKGFYPSDIAVEWESNGQPENNYKTTPPVLDSDGSFFLYSKLTVDKSRWQQGNVFSCSVMHEALHNHYTQKSLSLSPGK

SEQ ID NO: 361 - protein, 354 aa, Artificial Sequence
  PR007294 HC
EVQLVESGGGLVKPGGSLRLSCVASGFTFSDYYMSWFRQAPGKGLEWVSYISGSGTTIDYADSVKGRFTISRDNAKNSLYLQMNSLRAEDTAVYYCAREREPVAGTLDFDNWGQGTLVTVSSEPKSSDKTHTCPPCPAPELLGGPSVFLFPPKPKDTLMISRTPEVTCVVVDVSHEDPEVKFNWYVDGVEVHNAKTKPREEQYNSTYRVVSVLTVLHQDWLNGKEYKCKVSNKALPAPIEKTISKAKGQPREPQVYTLPPSREEMTKNQVSLTCLVKGFYPSDIAVEWESNGQPENNYKTTPPVLDSDGSFFLYSKLTVDKSRWQQGNVFSCSVMHEALHNHYTQKSLSLSPGK

SEQ ID NO: 362 - protein, 356 aa, Artificial Sequence
  PR007295 HC
EVQLVESGGGLVKPGGSLRLSCAASGFTFSDYYMSWIRQAPGKGLEWVSYISNNGSTIYYADSVKGRFTISRDNAKNSLYLQMNSLRAEDTAVYYCARVRPGGSGNYWDWFDPWGQGTMVTVSSEPKSSDKTHTCPPCPAPELLGGPSVFLFPPKPKDTLMISRTPEVTCVVVDVSHEDPEVKFNWYVDGVEVHNAKTKPREEQYNSTYRVVSVLTVLHQDWLNGKEYKCKVSNKALPAPIEKTISKAKGQPREPQVYTLPPSREEMTKNQVSLTCLVKGFYPSDIAVEWESNGQPENNYKTTPPVLDSDGSFFLYSKLTVDKSRWQQGNVFSCSVMHEALHNHYTQKSLSLSPGK

SEQ ID NO: 363 - protein, 354 aa, Artificial Sequence
  PR007296 HC
EVQLVESGGGLVKPGGSLRLSCVASGFTFSDYYMSWFRQAPGKGLEWVSYISGSGTTIDYADSVKGRFTISRDNAKNSLYLQMNSLRAEDTAVYYCAREREAVAGTLDFDNWGQGTPVTVSSEPKSSDKTHTCPPCPAPELLGGPSVFLFPPKPKDTLMISRTPEVTCVVVDVSHEDPEVKFNWYVDGVEVHNAKTKPREEQYNSTYRVVSVLTVLHQDWLNGKEYKCKVSNKALPAPIEKTISKAKGQPREPQVYTLPPSREEMTKNQVSLTCLVKGFYPSDIAVEWESNGQPENNYKTTPPVLDSDGSFFLYSKLTVDKSRWQQGNVFSCSVMHEALHNHYTQKSLSLSPGK

SEQ ID NO: 364 - protein, 356 aa, Artificial Sequence
  PR007297 HC
EVQLVESGGGLVKPGGSLRLSCAASGFTFSDYYMSWIRQAPGKGLEWVSYISRSGSTIYYADSVKGRFTISRDNAKNSLYLQMNSLRAEDTAVYYCARVRPGGSGNYWDWFDPWGQGTLVTVSSEPKSSDKTHTCPPCPAPELLGGPSVFLFPPKPKDTLMISRTPEVTCVVVDVSHEDPEVKFNWYVDGVEVHNAKTKPREEQYNSTYRVVSVLTVLHQDWLNGKEYKCKVSNKALPAPIEKTISKAKGQPREPQVYTLPPSREEMTKNQVSLTCLVKGFYPSDIAVEWESNGQPENNYKTTPPVLDSDGSFFLYSKLTVDKSRWQQGNVFSCSVMHEALHNHYTQKSLSLSPGK

SEQ ID NO: 365 - protein, 354 aa, Artificial Sequence
  PR007298 HC
EVQLVESGGGLVKPGGSLRLSCAASGFTFSDYYMSWVRQAPGKGLEWVSYISSSGSTIDYADSVKGRFTISRDNAKNSLFLEMNSLRAEDTAVYYCAREREEVAGTLDFDNWGQGTLVTVSSEPKSSDKTHTCPPCPAPELLGGPSVFLFPPKPKDTLMISRTPEVTCVVVDVSHEDPEVKFNWYVDGVEVHNAKTKPREEQYNSTYRVVSVLTVLHQDWLNGKEYKCKVSNKALPAPIEKTISKAKGQPREPQVYTLPPSREEMTKNQVSLTCLVKGFYPSDIAVEWESNGQPENNYKTTPPVLDSDGSFFLYSKLTVDKSRWQQGNVFSCSVMHEALHNHYTQKSLSLSPGK

SEQ ID NO: 366 - protein, 346 aa, Artificial Sequence
  PR007299 HC
EVQLVESGGGLVKPGGSLRLSCAASGFTFSDYQMSWLRQAPGKGLEWVSYISSSGRTIYYADSVKGRFTISRDNAKNSVSLQMNSLRAEDTAVYYCAREGRFFPGQGTPVTVSSEPKSSDKTHTCPPCPAPELLGGPSVFLFPPKPKDTLMISRTPEVTCVVVDVSHEDPEVKFNWYVDGVEVHNAKTKPREEQYNSTYRVVSVLTVLHQDWLNGKEYKCKVSNKALPAPIEKTISKAKGQPREPQVYTLPPSREEMTKNQVSLTCLVKGFYPSDIAVEWESNGQPENNYKTTPPVLDSDGSFFLYSKLTVDKSRWQQGNVFSCSVMHEALHNHYTQKSLSLSPGK

SEQ ID NO: 367 - protein, 356 aa, Artificial Sequence
  PR007300 HC
EVQLVESGGGLVKPGGSLRLSCTTSGFTFSDYYMNWVRQAPGKGLEWVSYISNNGSTIYYADSVKGRFTISRDNAKNSLYLQMNSLRAEDTAVYYCARVRPGGSGNYWDWFDPWGQGTPVTVSSEPKSSDKTHTCPPCPAPELLGGPSVFLFPPKPKDTLMISRTPEVTCVVVDVSHEDPEVKFNWYVDGVEVHNAKTKPREEQYNSTYRVVSVLTVLHQDWLNGKEYKCKVSNKALPAPIEKTISKAKGQPREPQVYTLPPSREEMTKNQVSLTCLVKGFYPSDIAVEWESNGQPENNYKTTPPVLDSDGSFFLYSKLTVDKSRWQQGNVFSCSVMHEALHNHYTQKSLSLSPGK

SEQ ID NO: 368 - protein, 356 aa, Artificial Sequence
  PR007381 HC
EVQLLESGGGLVQPGGSLRLSCAASGFTFSNYAMSWVRQAPGKGLEWVSSIDASGGDTYYADSVKGRFTISRDNSKNTLYLQMNSLRAEDTAVYYCAKEGSHGTDDSHYDVDVWGQGTTVTVSSEPKSCDKTHTCPPCPAPELLGGPSVFLFPPKPKDTLMISRTPEVTCVVVDVSHEDPEVKFNWYVDGVEVHNAKTKPREEQYNSTYRVVSVLTVLHQDWLNGKEYKCKVSNKALPAPIEKTISKAKGQPREPQVYTLPPSREEMTKNQVSLTCLVKGFYPSDIAVEWESNGQPENNYKTTPPVLDSDGSFFLYSKLTVDKSRWQQGNVFSCSVMHEALHNHYTQKSLSLSPGK

SEQ ID NO: 369 - protein, 578 aa, Artificial Sequence
  PR007130 Chain
EVQLVESGGGLVQPGGSLRLSCAASGFTFSSYWMSWVRQAPGKGLEWVANIKQEGSEKYYVDSVKGRFTISRDNAKNSLYLQMNSLRAEDTAVYYCARDRAVAGAFDIWGQGTMVTVSSASTKGPSVFPLAPSSKSTSGGTAALGCLVKDYFPEPVTVSWNSGALTSGVHTFPAVLQSSGLYSLSSVVTVPSSSLGTQTYICNVNHKPSNTKVDKKVEPKSCDKTHTCPPCPAPEAAGAPSVFLFPPKPKDTLMISRTPEVTCVVVDVSHEDPEVKFNWYVDGVEVHNAKTKPREEQYNSTYRVVSVLTVLHQDWLNGKEYKCKVSNKALPAPIEKTISKAKGQPREPQVYTLPPSREEMTKNQVSLTCLVKGFYPSDIAVEWESNGQPENNYKTTPPVLDSDGSFFLYSKLTVDKSRWQQGNVFSCSVMHEALHNHYTQKSLSLSPGGGSGGSEVQLLESGGGLVQPGGSLRLSCAASGFTFSNYAMSWFRQPPETGLKWVSSIDASGGDTYYADSVKGRFTISRDNSKNTLYLQMNSLRAEDTAVYYCAKEGSHGTDDSHYDVDVWGQGTTVTVSS

SEQ ID NO: 370 - protein, 576 aa, Artificial Sequence
  PR007132 Chain
EVQLVESGGGLVQPGGSLRLSCAASGFTFSSYWMSWVRQAPGKGLEWVANIKQEGSEKYYVDSVKGRFTISRDNAKNSLYLQMNSLRAEDTAVYYCARDRAVAGAFDIWGQGTMVTVSSASTKGPSVFPLAPSSKSTSGGTAALGCLVKDYFPEPVTVSWNSGALTSGVHTFPAVLQSSGLYSLSSVVTVPSSSLGTQTYICNVNHKPSNTKVDKKVEPKSCDKTHTCPPCPAPEAAGAPSVFLFPPKPKDTLMISRTPEVTCVVVDVSHEDPEVKFNWYVDGVEVHNAKTKPREEQYNSTYRVVSVLTVLHQDWLNGKEYKCKVSNKALPAPIEKTISKAKGQPREPQVYTLPPSREEMTKNQVSLTCLVKGFYPSDIAVEWESNGQPENNYKTTPPVLDSDGSFFLYSKLTVDKSRWQQGNVFSCSVMHEALHNHYTQKSLSLSPGGGSGGSEVQLVESGGGLVKPGGSLRLSCAASGFTFSDYYMSWIRQAPGKGLEWVSYISSSGSTIYYADSVKGRFTISRDNAKNSLYLQMNSLRAEDTAVYYCARVKPVAGTWDWFDPWGQGTPVTVSS

SEQ ID NO: 371 - protein, 576 aa, Artificial Sequence
  PR007133 Chain
EVQLVESGGGLVQPGGSLRLSCAASGFTFSSYWMSWVRQAPGKGLEWVANIKQEGSEKYYVDSVKGRFTISRDNAKNSLYLQMNSLRAEDTAVYYCARDRAVAGAFDIWGQGTMVTVSSASTKGPSVFPLAPSSKSTSGGTAALGCLVKDYFPEPVTVSWNSGALTSGVHTFPAVLQSSGLYSLSSVVTVPSSSLGTQTYICNVNHKPSNTKVDKKVEPKSCDKTHTCPPCPAPEAAGAPSVFLFPPKPKDTLMISRTPEVTCVVVDVSHEDPEVKFNWYVDGVEVHNAKTKPREEQYNSTYRVVSVLTVLHQDWLNGKEYKCKVSNKALPAPIEKTISKAKGQPREPQVYTLPPSREEMTKNQVSLTCLVKGFYPSDIAVEWESNGQPENNYKTTPPVLDSDGSFFLYSKLTVDKSRWQQGNVFSCSVMHEALHNHYTQKSLSLSPGGGSGGSEVQLEESGGGLVKPGGSLRLSCAASGFTFSDYYMSWFRQAPGKGLEWVSYISSSGSITDYADAVKGRFNISRDNAKNSLYLQMNSLRAEDTAVYYCAREREAVAGTLDFDNWGQGTLVTVSS

SEQ ID NO: 372 - protein, 576 aa, Artificial Sequence
  PR007135 Chain
EVQLVESGGGLVQPGGSLRLSCAASGFTFSSYWMSWVRQAPGKGLEWVANIKQEGSEKYYVDSVKGRFTISRDNAKNSLYLQMNSLRAEDTAVYYCARDRAVAGAFDIWGQGTMVTVSSASTKGPSVFPLAPSSKSTSGGTAALGCLVKDYFPEPVTVSWNSGALTSGVHTFPAVLQSSGLYSLSSVVTVPSSSLGTQTYICNVNHKPSNTKVDKKVEPKSCDKTHTCPPCPAPEAAGAPSVFLFPPKPKDTLMISRTPEVTCVVVDVSHEDPEVKFNWYVDGVEVHNAKTKPREEQYNSTYRVVSVLTVLHQDWLNGKEYKCKVSNKALPAPIEKTISKAKGQPREPQVYTLPPSREEMTKNQVSLTCLVKGFYPSDIAVEWESNGQPENNYKTTPPVLDSDGSFFLYSKLTVDKSRWQQGNVFSCSVMHEALHNHYTQKSLSLSPGGGSGGSEVQLVESGGGLVKPGGSLRLSCAASGFTFSDYYMSWFRQAPGKGLEWVSYISGSGSIIDYADSVKGRFTISRDNAKNSLYLQMNSLRAEDTAVYYCSREREAVAGTLDFDYWGQGTLVTVSS

SEQ ID NO: 373 - protein, 576 aa, Artificial Sequence
  PR007136 Chain
EVQLVESGGGLVQPGGSLRLSCAASGFTFSSYWMSWVRQAPGKGLEWVANIKQEGSEKYYVDSVKGRFTISRDNAKNSLYLQMNSLRAEDTAVYYCARDRAVAGAFDIWGQGTMVTVSSASTKGPSVFPLAPSSKSTSGGTAALGCLVKDYFPEPVTVSWNSGALTSGVHTFPAVLQSSGLYSLSSVVTVPSSSLGTQTYICNVNHKPSNTKVDKKVEPKSCDKTHTCPPCPAPEAAGAPSVFLFPPKPKDTLMISRTPEVTCVVVDVSHEDPEVKFNWYVDGVEVHNAKTKPREEQYNSTYRVVSVLTVLHQDWLNGKEYKCKVSNKALPAPIEKTISKAKGQPREPQVYTLPPSREEMTKNQVSLTCLVKGFYPSDIAVEWESNGQPENNYKTTPPVLDSDGSFFLYSKLTVDKSRWQQGNVFSCSVMHEALHNHYTQKSLSLSPGGGSGGSEVQLVESGGGLVKPGGSLRLSCAASGFTFSDYYMSWFRQAPGKGLEWVSYISSSGSTQDYADSVKGRFTISRDNAKNSLYLQMNSLRAEDTAVYYCAREREPVAGTLDFDNWGQGTPVTVSS

SEQ ID NO: 374 - protein, 576 aa, Artificial Sequence
  PR007137 Chain
EVQLVESGGGLVQPGGSLRLSCAASGFTFSSYWMSWVRQAPGKGLEWVANIKQEGSEKYYVDSVKGRFTISRDNAKNSLYLQMNSLRAEDTAVYYCARDRAVAGAFDIWGQGTMVTVSSASTKGPSVFPLAPSSKSTSGGTAALGCLVKDYFPEPVTVSWNSGALTSGVHTFPAVLQSSGLYSLSSVVTVPSSSLGTQTYICNVNHKPSNTKVDKKVEPKSCDKTHTCPPCPAPEAAGAPSVFLFPPKPKDTLMISRTPEVTCVVVDVSHEDPEVKFNWYVDGVEVHNAKTKPREEQYNSTYRVVSVLTVLHQDWLNGKEYKCKVSNKALPAPIEKTISKAKGQPREPQVYTLPPSREEMTKNQVSLTCLVKGFYPSDIAVEWESNGQPENNYKTTPPVLDSDGSFFLYSKLTVDKSRWQQGNVFSCSVMHEALHNHYTQKSLSLSPGGGSGGSEVQLVESGGGVVQPGRSLRLSCAASGFTFSDYYMSWFRQAPGKGLEWVSYISSSGTTIDYADSVKGRFTISRDNAKNSLYLQMNSLRAEDTAVYYCAREREEVAGTLDFDYWGQGTPVTVSS

SEQ ID NO: 375 - protein, 578 aa, Artificial Sequence
  PR007138 Chain
EVQLVESGGGLVQPGGSLRLSCAASGFTFSSYWMSWVRQAPGKGLEWVANIKQEGSEKYYVDSVKGRFTISRDNAKNSLYLQMNSLRAEDTAVYYCARDRAVAGAFDIWGQGTMVTVSSASTKGPSVFPLAPSSKSTSGGTAALGCLVKDYFPEPVTVSWNSGALTSGVHTFPAVLQSSGLYSLSSVVTVPSSSLGTQTYICNVNHKPSNTKVDKKVEPKSCDKTHTCPPCPAPEAAGAPSVFLFPPKPKDTLMISRTPEVTCVVVDVSHEDPEVKFNWYVDGVEVHNAKTKPREEQYNSTYRVVSVLTVLHQDWLNGKEYKCKVSNKALPAPIEKTISKAKGQPREPQVYTLPPSREEMTKNQVSLTCLVKGFYPSDIAVEWESNGQPENNYKTTPPVLDSDGSFFLYSKLTVDKSRWQQGNVFSCSVMHEALHNHYTQKSLSLSPGGGSGGSEVQLVESGGGLVKPGGSLRLSCVTSGFTFSDYYMNWIRQAPGKGQEWVSYISGNGSTIYYADSVKGRFTISRDNAKNSLYLQMNSLRAEDTAVYYCARVRPGGSGNYWDWFDPWGQGTPVTVSS

SEQ ID NO: 376 - protein, 576 aa, Artificial Sequence
  PR007139 Chain
EVQLVESGGGLVQPGGSLRLSCAASGFTFSSYWMSWVRQAPGKGLEWVANIKQEGSEKYYVDSVKGRFTISRDNAKNSLYLQMNSLRAEDTAVYYCARDRAVAGAFDIWGQGTMVTVSSASTKGPSVFPLAPSSKSTSGGTAALGCLVKDYFPEPVTVSWNSGALTSGVHTFPAVLQSSGLYSLSSVVTVPSSSLGTQTYICNVNHKPSNTKVDKKVEPKSCDKTHTCPPCPAPEAAGAPSVFLFPPKPKDTLMISRTPEVTCVVVDVSHEDPEVKFNWYVDGVEVHNAKTKPREEQYNSTYRVVSVLTVLHQDWLNGKEYKCKVSNKALPAPIEKTISKAKGQPREPQVYTLPPSREEMTKNQVSLTCLVKGFYPSDIAVEWESNGQPENNYKTTPPVLDSDGSFFLYSKLTVDKSRWQQGNVFSCSVMHEALHNHYTQKSLSLSPGGGSGGSEVQLVESGGGLVKPGGSLRLSCAASGFTFSDYYMSWIRQAPGKGLEWVSYISSSGSTIDYADSVKGRFTISRDNAKNSLYLQMNSLRAEDTAVYYCAREREEVAGTLDYDNWGQGTLVTVSS

SEQ ID NO: 377 - protein, 576 aa, Artificial Sequence
  PR007141 Chain
EVQLVESGGGLVQPGGSLRLSCAASGFTFSSYWMSWVRQAPGKGLEWVANIKQEGSEKYYVDSVKGRFTISRDNAKNSLYLQMNSLRAEDTAVYYCARDRAVAGAFDIWGQGTMVTVSSASTKGPSVFPLAPSSKSTSGGTAALGCLVKDYFPEPVTVSWNSGALTSGVHTFPAVLQSSGLYSLSSVVTVPSSSLGTQTYICNVNHKPSNTKVDKKVEPKSCDKTHTCPPCPAPEAAGAPSVFLFPPKPKDTLMISRTPEVTCVVVDVSHEDPEVKFNWYVDGVEVHNAKTKPREEQYNSTYRVVSVLTVLHQDWLNGKEYKCKVSNKALPAPIEKTISKAKGQPREPQVYTLPPSREEMTKNQVSLTCLVKGFYPSDIAVEWESNGQPENNYKTTPPVLDSDGSFFLYSKLTVDKSRWQQGNVFSCSVMHEALHNHYTQKSLSLSPGGGSGGSEVQLVESGGGLVKPGGSLRLSCVASGFTFSDYYMSWFRQAPGKGLEWVSYISGSGTTIDYADSVKGRFTISRDNAKNSLYLQMNSLRAEDTAVYYCAREREPVAGTLDFDNWGQGTLVTVSS

SEQ ID NO: 378 - protein, 578 aa, Artificial Sequence
  PR007142 Chain
EVQLVESGGGLVQPGGSLRLSCAASGFTFSSYWMSWVRQAPGKGLEWVANIKQEGSEKYYVDSVKGRFTISRDNAKNSLYLQMNSLRAEDTAVYYCARDRAVAGAFDIWGQGTMVTVSSASTKGPSVFPLAPSSKSTSGGTAALGCLVKDYFPEPVTVSWNSGALTSGVHTFPAVLQSSGLYSLSSVVTVPSSSLGTQTYICNVNHKPSNTKVDKKVEPKSCDKTHTCPPCPAPEAAGAPSVFLFPPKPKDTLMISRTPEVTCVVVDVSHEDPEVKFNWYVDGVEVHNAKTKPREEQYNSTYRVVSVLTVLHQDWLNGKEYKCKVSNKALPAPIEKTISKAKGQPREPQVYTLPPSREEMTKNQVSLTCLVKGFYPSDIAVEWESNGQPENNYKTTPPVLDSDGSFFLYSKLTVDKSRWQQGNVFSCSVMHEALHNHYTQKSLSLSPGGGSGGSEVQLVESGGGLVKPGGSLRLSCAASGFTFSDYYMSWIRQAPGKGLEWVSYISNNGSTIYYADSVKGRFTISRDNAKNSLYLQMNSLRAEDTAVYYCARVRPGGSGNYWDWFDPWGQGTMVTVSS

SEQ ID NO: 379 - protein, 576 aa, Artificial Sequence
  PR007143 Chain
EVQLVESGGGLVQPGGSLRLSCAASGFTFSSYWMSWVRQAPGKGLEWVANIKQEGSEKYYVDSVKGRFTISRDNAKNSLYLQMNSLRAEDTAVYYCARDRAVAGAFDIWGQGTMVTVSSASTKGPSVFPLAPSSKSTSGGTAALGCLVKDYFPEPVTVSWNSGALTSGVHTFPAVLQSSGLYSLSSVVTVPSSSLGTQTYICNVNHKPSNTKVDKKVEPKSCDKTHTCPPCPAPEAAGAPSVFLFPPKPKDTLMISRTPEVTCVVVDVSHEDPEVKFNWYVDGVEVHNAKTKPREEQYNSTYRVVSVLTVLHQDWLNGKEYKCKVSNKALPAPIEKTISKAKGQPREPQVYTLPPSREEMTKNQVSLTCLVKGFYPSDIAVEWESNGQPENNYKTTPPVLDSDGSFFLYSKLTVDKSRWQQGNVFSCSVMHEALHNHYTQKSLSLSPGGGSGGSEVQLVESGGGLVKPGGSLRLSCVASGFTFSDYYMSWFRQAPGKGLEWVSYISGSGTTIDYADSVKGRFTISRDNAKNSLYLQMNSLRAEDTAVYYCAREREAVAGTLDFDNWGQGTPVTVSS

SEQ ID NO: 380 - protein, 578 aa, Artificial Sequence
  PR007145 Chain
EVQLVESGGGLVQPGGSLRLSCAASGFTFSSYWMSWVRQAPGKGLEWVANIKQEGSEKYYVDSVKGRFTISRDNAKNSLYLQMNSLRAEDTAVYYCARDRAVAGAFDIWGQGTMVTVSSASTKGPSVFPLAPSSKSTSGGTAALGCLVKDYFPEPVTVSWNSGALTSGVHTFPAVLQSSGLYSLSSVVTVPSSSLGTQTYICNVNHKPSNTKVDKKVEPKSCDKTHTCPPCPAPEAAGAPSVFLFPPKPKDTLMISRTPEVTCVVVDVSHEDPEVKFNWYVDGVEVHNAKTKPREEQYNSTYRVVSVLTVLHQDWLNGKEYKCKVSNKALPAPIEKTISKAKGQPREPQVYTLPPSREEMTKNQVSLTCLVKGFYPSDIAVEWESNGQPENNYKTTPPVLDSDGSFFLYSKLTVDKSRWQQGNVFSCSVMHEALHNHYTQKSLSLSPGGGSGGSEVQLVESGGGLVKPGGSLRLSCAASGFTFSDYYMSWIRQAPGKGLEWVSYISRSGSTIYYADSVKGRFTISRDNAKNSLYLQMNSLRAEDTAVYYCARVRPGGSGNYWDWFDPWGQGTLVTVSS

SEQ ID NO: 381 - protein, 576 aa, Artificial Sequence
  PR007146 Chain
EVQLVESGGGLVQPGGSLRLSCAASGFTFSSYWMSWVRQAPGKGLEWVANIKQEGSEKYYVDSVKGRFTISRDNAKNSLYLQMNSLRAEDTAVYYCARDRAVAGAFDIWGQGTMVTVSSASTKGPSVFPLAPSSKSTSGGTAALGCLVKDYFPEPVTVSWNSGALTSGVHTFPAVLQSSGLYSLSSVVTVPSSSLGTQTYICNVNHKPSNTKVDKKVEPKSCDKTHTCPPCPAPEAAGAPSVFLFPPKPKDTLMISRTPEVTCVVVDVSHEDPEVKFNWYVDGVEVHNAKTKPREEQYNSTYRVVSVLTVLHQDWLNGKEYKCKVSNKALPAPIEKTISKAKGQPREPQVYTLPPSREEMTKNQVSLTCLVKGFYPSDIAVEWESNGQPENNYKTTPPVLDSDGSFFLYSKLTVDKSRWQQGNVFSCSVMHEALHNHYTQKSLSLSPGGGSGGSEVQLVESGGGLVKPGGSLRLSCAASGFTFSDYYMSWVRQAPGKGLEWVSYISSSGSTIDYADSVKGRFTISRDNAKNSLFLEMNSLRAEDTAVYYCAREREEVAGTLDFDNWGQGTLVTVSS

SEQ ID NO: 382 - protein, 578 aa, Artificial Sequence
  PR007149 Chain
EVQLVESGGGLVQPGGSLRLSCAASGFTFSSYWMSWVRQAPGKGLEWVANIKQEGSEKYYVDSVKGRFTISRDNAKNSLYLQMNSLRAEDTAVYYCARDRAVAGAFDIWGQGTMVTVSSASTKGPSVFPLAPSSKSTSGGTAALGCLVKDYFPEPVTVSWNSGALTSGVHTFPAVLQSSGLYSLSSVVTVPSSSLGTQTYICNVNHKPSNTKVDKKVEPKSCDKTHTCPPCPAPEAAGAPSVFLFPPKPKDTLMISRTPEVTCVVVDVSHEDPEVKFNWYVDGVEVHNAKTKPREEQYNSTYRVVSVLTVLHQDWLNGKEYKCKVSNKALPAPIEKTISKAKGQPREPQVYTLPPSREEMTKNQVSLTCLVKGFYPSDIAVEWESNGQPENNYKTTPPVLDSDGSFFLYSKLTVDKSRWQQGNVFSCSVMHEALHNHYTQKSLSLSPGGGSGGSEVQLVESGGGLVKPGGSLRLSCTTSGFTFSDYYMNWVRQAPGKGLEWVSYISNNGSTIYYADSVKGRFTISRDNAKNSLYLQMNSLRAEDTAVYYCARVRPGGSGNYWDWFDPWGQGTPVTVSS